European Patent Application EP 4 378 476 A1, published June 5, 2024. Title: PHARMACEUTICAL COMPOSITION FOR TREATMENT AND/OR PREVENTION OF CANCER. Applicant: TORAY Industries, Inc. The sequence listing filed with the application follows.

SEQUENCE LISTING (324 sequences)

SEQ ID NO: 1 - DNA, 5562 bp, Homo sapiens
  source 1..5562: mol_type = other DNA
  CDS 190..2319: protein_id = 310; translation = MPSATSHSGSGSKSSGPPPPSGSSGSEAAAGAGAAAPASQHPATGTGAVQTEAMKQILGVIDKKLRNLEKKKGKLDDYQERMNKGERLNQDQLDAVSKYQEVTNNLEFAKELQRSFMALSQDIQKTIKKTARREQLMREEAEQKRLKTVLELQYVLDKLGDDEVRTDLKQGLNGVPILSEEELSLLDEFYKLVDPERDMSLRLNEQYEHASIHLWDLLEGKEKPVCGTTYKVLKEIVERVFQSNYFDSTHNHQNGLCEEEEAASAPAVEDQVPEAEPEPAEEYTEQSEVESTEYVNRQFMAETQFTSGEKEQVDEWTVETVEVVNSLQQQPQAASPSVPEPHSLTPVAQADPLVRRQRVQDLMAQMQGPYNFIQDSMLDFENQTLDPAIVSAQPMNPTQNMDMPQLVCPPVHSESRLAQPNQVPVQPEATQVPLVSSTSEGYTASQPLYQPSHATEQRPQKEPIDQIQATISLNTDQTTASSSLPAASQPQVFQAGTSKPLHSSGINVNAAPFQSMQTVFNMNAPVPPVNEPETLKQQNQYQASYNQSFSSQPHQVEQTELQQEQLQTVVGTYHGSPDQSHQVTGNHQQPPQQNTGFPRSNQPYYNSRGVSRGGSRGARGLMNGYRGPANGFRGGYDGYRPSFSNTPNSGYTQSQFSAPRDYSGYQRDGYQQNFKRGSGQSGPRGAPRGRGGPPRPNRGMPQMNTQQVN
cagagggctgctggctggctaagtccctcccgctcccggctctcgcctcactaggagcggctctcggtgcagcgggacagggcgaagcggcctgcgcccacggagcgcgcgacactgcccggaagggaccgccacccttgccccctcagctgcccactcgtgatttccagcggcctccgcgcgcgcacgatgccctcggccaccagccacagcgggagcggcagcaagtcgtccggaccgccaccgccgtcgggttcctccgggagtgaggcggccgcgggagccggggccgccgcgccggcttctcagcaccccgcaaccggcaccggcgctgtccagaccgaggccatgaagcagattctcggggtgatcgacaagaaacttcggaacctggagaagaaaaagggtaagcttgatgattaccaggaacgaatgaacaaaggggaaaggcttaatcaagatcagctggatgccgtttctaagtaccaggaagtcacaaataatttggagtttgcaaaagaattacagaggagtttcatggcactaagtcaagatattcagaaaacaataaagaagacagcacgtcgggagcagcttatgagagaagaagctgaacagaaacgtttaaaaactgtacttgagctacagtatgttttggacaaattgggagatgatgaagtgcggactgacctgaaacaaggtttgaatggagtgccaatattgtccgaagaggagttgtcattgttggatgaattctataagctagtagaccctgaacgggacatgagcttgaggttgaatgaacagtatgaacatgcctccattcacctgtgggacctgctggaagggaaggaaaaacctgtatgtggaaccacctataaagttctaaaggaaattgttgagcgtgtttttcagtcaaactactttgacagcacccacaaccaccagaatgggctgtgtgaggaagaagaggcagcctcagcacctgcagttgaagaccaggtacctgaagctgaacctgagccagcagaagagtacactgagcaaagtgaagttgaatcaacagagtatgtaaatagacagttcatggcagaaacacagttcaccagtggtgaaaaggagcaggtagatgagtggacagttgaaacggttgaggtggtaaattcactccagcagcaacctcaggctgcatccccttcagtaccagagccccactctttgactccagtggctcaggcagatccccttgtgagaagacagcgagtacaagaccttatggcacaaatgcagggtccctataatttcatacaggattcaatgctggattttgaaaatcagacacttgatcctgccattgtatctgcacagcctatgaatccaacacaaaacatggacatgccccagctggtttgccctccagttcattctgaatctagacttgctcagcctaatcaagttcctgtacaaccagaagcgacacaggttcctttggtatcatccacaagtgaggggtacacagcatctcaacccttgtaccagccttctcatgctacagagcaacgaccacagaaggaaccaattgatcagattcaggcaacaatctctttaaatacagaccagactacagcatcatcatcccttcctgctgcgtctcagcctcaagtatttcaggctgggacaagcaaacctttacatagcagtggaatcaatgtaaatgcagctccattccaatccatgcaaacggtgttcaatatgaatgccccagttcctcctgttaatgaaccagaaactttaaaacagcaaaatcagtaccaggccagttataaccagagcttttctagtcagcctcaccaagtagaacaaacagagcttcagcaagaacagcttcaaacagtggttggcacttaccatggttccccagaccagtcccatcaagtgactggtaaccaccagcagcctcctcagcagaacactggatttccacgtagcaatcagccctattacaatagtcgtggtgtgtctcgtggaggctcccgtggtgctagaggcttgatgaatggataccggggccctgccaatggattcagaggaggatatgatggttaccgcccttcattctctaacactccaaacagtggttatacacagtctcagttcagtgctccccgggattactctggctatcaacgggatggatatcagcagaatttcaagcgaggctctgggcagagtggaccacggggagccccacgaggtcgtggagggcccccaagacccaacagagggatgccgcaaatgaacactcagcaagtgaattaatctgattcacaggattatgtttaatcgccaaaaacacactggccagtgtaccataatatgttaccagaagagttattatctatttgttctccctttcaggaaacttattgtaaagggactgttttcatcccataaagacaggactacaattgtcagctttctattacctggatatggaaggaaactatttttactctgcatgttctgtcctaagcgtcatcttgagccttgcacatgatactcagattcctcacccttgcttaggagtaaaacaatatactttacagggtgataataatctccatagttatttgaagtggcttgaaaaaggcaagattgacttttatgacattggataaaatctacaaatcagccctcgagttattcaatgataactgacaaactaaattatttccctagaaaggaagatgaaaggagtggagtgtggtttggcagaacaactgcatttcacagcttttccagttaaattggagcactgaacgttcagatgcataccaaattatgcatgggtcctaatcacacatataaggctggctaccagctttgacacagcactgttcatctggccaaacaactgtggttaaaaacacatgtaaaatgctttttaacagctgatactgtataagacaaagccaagatgcaaaattaggctttgattggcactttttgaaaaatatgcaacaaatatgggatgtaatccggatggccgcttctgtacttaatgtgaaatatttagatacctttttgaacacttaacagtttctttgagacaatgacttttgtaaggattggtactatctatcattccttatgacatgtacattgtctgtcactaatccttggattttgctgtattgtcacctaaattggtacaggtactgatgaaaatctctagtggataatcataacactctcggtcacatgtttttccttcagcttgaaagcttttttttaaaaggaaaagataccaaatgcctgctgctaccacccttttcaattgctatcttttgaaaggcaccagtatgtgttttagattgatttccctgtttcagggaaatcacggacagtagtttcagttctgatggtataagcaaaacaaataaaacgtttataaaagttgtatcttgaaacactggtgttcaacagctagcagcttatgtgattcaccccatgccacgttagtgtcacaaattttatggtttatctccagcaacatttctctagtacttgcacttattatcttttgtctaatttaaccttaactgaattctccgtttctcctggaggcatttatattcagtgataattccttcccttagatgcatagggagagtctctaaatttgatggaaatggacacttgagtagtgacttagccttatgtactctgttggaatttgtgctagcagtttgagcactagttctgtgtgcctaggaagttaatgctgcttattgtctcattctgacttcatggagaattaatcccacctttaagcaaaggctactaagttaatggtattttctgtgcagaaattaaattttattttcagcatttagcccaggaattcttccagtaggtgctcagctatttaaaaacaaaactattctcaaacattcatcattagacaactggagtttttgctggttttgtaacctaccaaaatggataggctgttgaacattccacattcaaaagttttgtagggtggtgggaaatgggggatcttcaatgtttattttaaaataaaataaaataagttcttgacttttctcatgtgtggttgtggtacatcatattggaagggttaacctgttactttggcaaatgagtatttttttgctagcacctccccttgcgtgctttaaatgacatctgcctgggatgtaccacaaccatatgttacctgtatcttaggggaatggataaaatatttgtggtttactgggtaatccctagatgatgtatgcttgcagtcctatataaaactaaatttgctatctgtgtagaaaataatttcatgacatttacaatcaggactgaagtaagttcttcacacagtgacctctgaatcagtttcagagaagggatgggggagaaaatgccttctaggttttgaacttctatgcattagtgcagatgttgtgaatgtgtaaaggtgttcatagtttgactgtttctatgtatgttttttcaaagaattgttcctttttttgaactataatttttctttttttggttattttaccatcacagtttaaatgtatatcttttatgtctctactcagaccatatttttaaaggggtgcctcattatggggcagagaacttttcaataagtctcattaagatctgaatcttggttctaagcattctgtataatatgtgattgcttgtcctagctgcagaaggccttttgtttggtcaaatgcatattttagcagagtttcaaggaaatgattgtcacacatgtcactgtagcctcttggtgtagcaagctcacatacaaaatacttttgtatatgcataatataaatcatctcatgtggatatgaaacttcttttttaaaacttaaaaaggtagaatgttattgattaccttgattagggcagttttatttccagatcctaataattcctaaaaaatatggaaaagttttttttcaatcattgtaccttgatattaaaacaaatatcctttaagtatttctaatcagttagcttctacagttcttttgtctccttttatatgcagctcttacgtgggagacttttccacttaaaggagacatagaatgtgtgcttattctcagaaggttcattaactgaggtgatgagttaacaactagttgagcagtcagcttcctaagtgttttaggacatttgttcattatattttccgtcatataactagaggaagtggaatgcagataagtgccgaattcaaacccttcattttatgtttaagctcctgaatctgcattccacttgggttgtttttaagcattctaaattttagttgattataagttagatttcacagaatcagtattgcccttgatcttgtcctttttatggagttaacggggaggaagacccctcaggaaaacgaaagtaaattgttaaggctcatcttcatacctttttccattttgaatcctacaaaaatactgcaaaagactagtgaatgtttaaaattacactagattaaataatatgaaagtc

SEQ ID NO: 2 - protein, 709 aa, Homo sapiens
MPSATSHSGSGSKSSGPPPPSGSSGSEAAAGAGAAAPASQHPATGTGAVQTEAMKQILGVIDKKLRNLEKKKGKLDDYQERMNKGERLNQDQLDAVSKYQEVTNNLEFAKELQRSFMALSQDIQKTIKKTARREQLMREEAEQKRLKTVLELQYVLDKLGDDEVRTDLKQGLNGVPILSEEELSLLDEFYKLVDPERDMSLRLNEQYEHASIHLWDLLEGKEKPVCGTTYKVLKEIVERVFQSNYFDSTHNHQNGLCEEEEAASAPAVEDQVPEAEPEPAEEYTEQSEVESTEYVNRQFMAETQFTSGEKEQVDEWTVETVEVVNSLQQQPQAASPSVPEPHSLTPVAQADPLVRRQRVQDLMAQMQGPYNFIQDSMLDFENQTLDPAIVSAQPMNPTQNMDMPQLVCPPVHSESRLAQPNQVPVQPEATQVPLVSSTSEGYTASQPLYQPSHATEQRPQKEPIDQIQATISLNTDQTTASSSLPAASQPQVFQAGTSKPLHSSGINVNAAPFQSMQTVFNMNAPVPPVNEPETLKQQNQYQASYNQSFSSQPHQVEQTELQQEQLQTVVGTYHGSPDQSHQVTGNHQQPPQQNTGFPRSNQPYYNSRGVSRGGSRGARGLMNGYRGPANGFRGGYDGYRPSFSNTPNSGYTQSQFSAPRDYSGYQRDGYQQNFKRGSGQSGPRGAPRGRGGPPRPNRGMPQMNTQQVN

SEQ ID NO: 3 - DNA, 3553 bp, Homo sapiens
  source 1..3553: mol_type = other DNA
  CDS 190..2274: protein_id = 311; translation = MPSATSHSGSGSKSSGPPPPSGSSGSEAAAGAGAAAPASQHPATGTGAVQTEAMKQILGVIDKKLRNLEKKKGKLDDYQERMNKGERLNQDQLDAVSKYQEVTNNLEFAKELQRSFMALSQDIQKTIKKTARREQLMREEAEQKRLKTVLELQYVLDKLGDDEVRTDLKQGLNGVPILSEEELSLLDEFYKLVDPERDMSLRLNEQYEHASIHLWDLLEGKEKPVCGTTYKVLKEIVERVFQSNYFDSTHNHQNGLCEEEEAASAPAVEDQVPEAEPEPAEEYTEQSEVESTEYVNRQFMAETQFTSGEKEQVDEWTVETVEVVNSLQQQPQAASPSVPEPHSLTPVAQADPLVRRQRVQDLMAQMQGPYNFIQDSMLDFENQTLDPAIVSAQPMNPTQNMDMPQLVCPPVHSESRLAQPNQVPVQPEATQVPLVSSTSEGYTASQPLYQPSHATEQRPQKEPIDQIQATISLNTDQTTASSSLPAASQPQVFQAGTSKPLHSSGINVNAAPFQSMQTVFNMNAPVPPVNEPETLKQQNQYQASYNQSFSSQPHQVEQTELQQEQLQTVVGTYHGSPDQSHQVTGNHQQPPQQNTGFPRSNQPYYNSRGVSRGGSRGARGLMNGYRGPANGFRGGYDGYRPSFSNTPNSGYTQSQFSAPRDYSGYQRDGYQQNFKRGSGQSGPRGAPRGNILWW
cagagggctgctggctggctaagtccctcccgctcccggctctcgcctcactaggagcggctctcggtgcagcgggacagggcgaagcggcctgcgcccacggagcgcgcgacactgcccggaagggaccgccacccttgccccctcagctgcccactcgtgatttccagcggcctccgcgcgcgcacgatgccctcggccaccagccacagcgggagcggcagcaagtcgtccggaccgccaccgccgtcgggttcctccgggagtgaggcggccgcgggagccggggccgccgcgccggcttctcagcaccccgcaaccggcaccggcgctgtccagaccgaggccatgaagcagattctcggggtgatcgacaagaaacttcggaacctggagaagaaaaagggtaagcttgatgattaccaggaacgaatgaacaaaggggaaaggcttaatcaagatcagctggatgccgtttctaagtaccaggaagtcacaaataatttggagtttgcaaaagaattacagaggagtttcatggcactaagtcaagatattcagaaaacaataaagaagacagcacgtcgggagcagcttatgagagaagaagctgaacagaaacgtttaaaaactgtacttgagctacagtatgttttggacaaattgggagatgatgaagtgcggactgacctgaaacaaggtttgaatggagtgccaatattgtccgaagaggagttgtcattgttggatgaattctataagctagtagaccctgaacgggacatgagcttgaggttgaatgaacagtatgaacatgcctccattcacctgtgggacctgctggaagggaaggaaaaacctgtatgtggaaccacctataaagttctaaaggaaattgttgagcgtgtttttcagtcaaactactttgacagcacccacaaccaccagaatgggctgtgtgaggaagaagaggcagcctcagcacctgcagttgaagaccaggtacctgaagctgaacctgagccagcagaagagtacactgagcaaagtgaagttgaatcaacagagtatgtaaatagacagttcatggcagaaacacagttcaccagtggtgaaaaggagcaggtagatgagtggacagttgaaacggttgaggtggtaaattcactccagcagcaacctcaggctgcatccccttcagtaccagagccccactctttgactccagtggctcaggcagatccccttgtgagaagacagcgagtacaagaccttatggcacaaatgcagggtccctataatttcatacaggattcaatgctggattttgaaaatcagacacttgatcctgccattgtatctgcacagcctatgaatccaacacaaaacatggacatgccccagctggtttgccctccagttcattctgaatctagacttgctcagcctaatcaagttcctgtacaaccagaagcgacacaggttcctttggtatcatccacaagtgaggggtacacagcatctcaacccttgtaccagccttctcatgctacagagcaacgaccacagaaggaaccaattgatcagattcaggcaacaatctctttaaatacagaccagactacagcatcatcatcccttcctgctgcgtctcagcctcaagtatttcaggctgggacaagcaaacctttacatagcagtggaatcaatgtaaatgcagctccattccaatccatgcaaacggtgttcaatatgaatgccccagttcctcctgttaatgaaccagaaactttaaaacagcaaaatcagtaccaggccagttataaccagagcttttctagtcagcctcaccaagtagaacaaacagagcttcagcaagaacagcttcaaacagtggttggcacttaccatggttccccagaccagtcccatcaagtgactggtaaccaccagcagcctcctcagcagaacactggatttccacgtagcaatcagccctattacaatagtcgtggtgtgtctcgtggaggctcccgtggtgctagaggcttgatgaatggataccggggccctgccaatggattcagaggaggatatgatggttaccgcccttcattctctaacactccaaacagtggttatacacagtctcagttcagtgctccccgggattactctggctatcaacgggatggatatcagcagaatttcaagcgaggctctgggcagagtggaccacggggagccccacgaggtaatattttgtggtggtgatcctagctcctaagtggagcttctgttctggccttggaagagctgttaatagtctgcatgttaggaatacatttatcctttccagacttgttgctagggattaaatgaaatgctctgtttctaaaacttaatcttggacccaaattttaatttttgaatgatttaattttccctgttactatataaactgtcttgaaaactagaacatattctcttctcagaaaaagtgtttttccaactgaaaattatttttcaggtcctaaaacctgctaaatgtttttaggaagtacttactgaaacatttttgtaagacatttttggaatgagattgaacatttatataaatttattattcctctttcatttttttgaaacatgcctattatattttagggccagacaccctttaatggccggataagccatagttaacatttagagaaccatttagaagtgatagaactaatggaatttgcaatgccttttggacctctattagtgatataaatatcaagttatttctgacttttaaacaaaactcccaaattcctaacttattgagctatacttaaaaaaaattacaggtttagagagttttttgtttttcttttactgttggaaaactacttcccattttggcaggaagttaacctatttaacaattagagctagcatttcatgtagtctgaaattctaaatggttctctgatttgagggaggttaaacatcaaacaggtttcctctattggccataacatgtataaaatgtgtgttaaggaggaattacaacgtactttgatttgaatactagtagaaactggccaggaaaaaggtacatttttctaaaaattaatggatcacttgggaattactgacttgactagaagtatcaaaggatgtttgcatgtgaatgtgggttatgttctttcccaccttgtagcatattcgatgaaagttgagttaactgatagctaaaaatctgttttaacagcatgtaaaaagttattttatctgttaaaagtcattatacagttttgaatgttatgtagtttctttttaacagtttaggtaataaggtctgttttcattctggtgcttttattaattttgatagtatgatgttacttactactgaaatgtaagctagagtgtacactagaatgtaagctccatgagagcaggtaccttgtctgtcttctctgctgtatctattcccaacgcttgatgatggtgcctggcacatagtaggcactcaataaatatttgttgaatgaatgaa

SEQ ID NO: 4 - protein, 694 aa, Homo sapiens
MPSATSHSGSGSKSSGPPPPSGSSGSEAAAGAGAAAPASQHPATGTGAVQTEAMKQILGVIDKKLRNLEKKKGKLDDYQERMNKGERLNQDQLDAVSKYQEVTNNLEFAKELQRSFMALSQDIQKTIKKTARREQLMREEAEQKRLKTVLELQYVLDKLGDDEVRTDLKQGLNGVPILSEEELSLLDEFYKLVDPERDMSLRLNEQYEHASIHLWDLLEGKEKPVCGTTYKVLKEIVERVFQSNYFDSTHNHQNGLCEEEEAASAPAVEDQVPEAEPEPAEEYTEQSEVESTEYVNRQFMAETQFTSGEKEQVDEWTVETVEVVNSLQQQPQAASPSVPEPHSLTPVAQADPLVRRQRVQDLMAQMQGPYNFIQDSMLDFENQTLDPAIVSAQPMNPTQNMDMPQLVCPPVHSESRLAQPNQVPVQPEATQVPLVSSTSEGYTASQPLYQPSHATEQRPQKEPIDQIQATISLNTDQTTASSSLPAASQPQVFQAGTSKPLHSSGINVNAAPFQSMQTVFNMNAPVPPVNEPETLKQQNQYQASYNQSFSSQPHQVEQTELQQEQLQTVVGTYHGSPDQSHQVTGNHQQPPQQNTGFPRSNQPYYNSRGVSRGGSRGARGLMNGYRGPANGFRGGYDGYRPSFSNTPNSGYTQSQFSAPRDYSGYQRDGYQQNFKRGSGQSGPRGAPRGNILWW

SEQ ID NO: 5 - DNA, 1605 bp, Canis familiaris
  source 1..1605: mol_type = other DNA
  CDS 46..1392: protein_id = 312; translation = MALSQDIQKTIKKTARREQLMREEAEQKRLKTVLELQYVLDKLGDDEVRTDLKQGLNGVPILSEEELSLLDEFYKLADPERDMSLRLNEQYEHASIHLWDLLEGKEKSVCGTTYKALKEIVERVFQSNYFDSTHNHQNGLCEEEEAASAPTVEDQVAEAEPEPAEEYTEQSEVESTEYVNRQFMAETQFSSGEKEQVDEWTVETVEVVNSLQQQPQAASPSVPEPHSLTPVAQADPLVRRQRVQDLMAQMQGPYNFIQDSMLDFENQTLDPAIVSAQPMNPTQNMDMPQLVCPPVHSESRLAQPNQVPVQPEATQVPLVSSTSEGYTASQPLYQPSHATEQRPQKEPIDQIQATISLNTDQTTASSSLPAASQPQVFQAGTSKPLHSSGINVNAAPFQSMQTVFNMNAPVPPVNEPETLKQQNQYQASYNQSFSSQPHQVEQTEGCRK
gtcacaaataacttggagtttgcaaaagaattacagaggagtttcatggcattaagtcaagatattcagaaaacaataaagaagactgcacgtcgggagcagcttatgagagaggaagcggaacaaaaacgtttaaaaactgtacttgagctccagtatgttttggacaaattgggagatgatgaagtgagaactgacctgaagcaaggtttgaatggagtgccaatattgtctgaagaagaattgtcgttgttggatgaattctacaaattagcagaccctgaacgggacatgagcttgaggttgaatgagcagtatgaacatgcttccattcacctgtgggacttgctggaaggaaaggaaaagtctgtatgtggaacaacctataaagcactaaaggaaattgttgagcgtgttttccagtcaaattactttgacagcactcacaaccaccagaatgggctatgtgaggaagaagaggcagcctcagcacctacagttgaagaccaggtagctgaagctgagcctgagccagcagaagaatacactgaacaaagtgaagttgaatcaacagagtatgtaaatagacaatttatggcagaaacacagttcagcagtggtgaaaaggagcaggtagatgagtggacggtcgaaacagtggaggtggtgaattcactccagcagcaacctcaggctgcgtctccttcagtaccagagccccactctttgactccggtggctcaggcagatccccttgtgagaagacagcgagtccaggaccttatggcgcagatgcaggggccctataatttcatacaggattcaatgctggattttgaaaaccagacactcgatcctgccattgtatctgcacagcctatgaatccgacacaaaacatggacatgccccagctggtttgccctccagttcattctgaatctagacttgctcaacctaatcaagttcctgtacaaccagaagctacacaggttcctttggtttcatccacaagtgaggggtatacagcatctcaacccttgtaccagccttctcatgctacagagcaacgaccacaaaaggaaccaattgaccagattcaggcaacaatctctttaaatacagaccagactacagcgtcatcatcccttccggctgcttctcagcctcaggtattccaggctgggacaagcaaaccattacatagcagtggaatcaatgtaaatgcagctccattccaatccatgcaaacggtgttcaatatgaatgccccagttcctcctgttaatgaaccagaaactttgaaacaacaaaatcagtaccaggccagttataaccagagcttttctagtcagcctcaccaagtagaacaaacagagggatgccgcaaatgaacactcagcaagtgaattaatctgattcacaggattatgtttaaacgccaaaaacacactggccagtgtaccataatatgttaccagaagagttattatctatttgttctccctttcaggaaacttattgtaaagggactgttttcatcccataaagacaggactacaattgtcagctttatattacctggaaaaaaaaaaaaaaaaaaaaaa

SEQ ID NO: 6 - protein, 448 aa, Canis familiaris
MALSQDIQKTIKKTARREQLMREEAEQKRLKTVLELQYVLDKLGDDEVRTDLKQGLNGVPILSEEELSLLDEFYKLADPERDMSLRLNEQYEHASIHLWDLLEGKEKSVCGTTYKALKEIVERVFQSNYFDSTHNHQNGLCEEEEAASAPTVEDQVAEAEPEPAEEYTEQSEVESTEYVNRQFMAETQFSSGEKEQVDEWTVETVEVVNSLQQQPQAASPSVPEPHSLTPVAQADPLVRRQRVQDLMAQMQGPYNFIQDSMLDFENQTLDPAIVSAQPMNPTQNMDMPQLVCPPVHSESRLAQPNQVPVQPEATQVPLVSSTSEGYTASQPLYQPSHATEQRPQKEPIDQIQATISLNTDQTTASSSLPAASQPQVFQAGTSKPLHSSGINVNAAPFQSMQTVFNMNAPVPPVNEPETLKQQNQYQASYNQSFSSQPHQVEQTEGCRK

SEQ ID NO: 7 - DNA, 4154 bp, Canis familiaris
  source 1..4154: mol_type = other DNA
  CDS 1..2154: protein_id = 313; translation = MPSATSLSGSGSKSSGPPPPSGSSGSEAAAAAGAAGAAGAGAAAPASQHPATGTGAVQTEAMKQILGVIDKKLRNLEKKKGKLDDYQERMNKGERLNQDQLDAVSKYQEVTNNLEFAKELQRSFMALSQDIQKTIKKTARREQLMREEAEQKRLKTVLELQYVLDKLGDDEVRTDLKQGLNGVPILSEEELSLLDEFYKLADPERDMSLRLNEQYEHASIHLWDLLEGKEKSVCGTTYKALKEIVERVFQSNYFDSTHNHQNGLCEEEEAASAPTVEDQVAEAEPEPAEEYTEQSEVESTEYVNRQFMAETQFSSGEKEQVDEWTVETVEVVNSLQQQPQAASPSVPEPHSLTPVAQADPLVRRQRVQDLMAQMQGPYNFIQDSMLDFENQTLDPAIVSAQPMNPTQNMDMPQLVCPPVHSESRLAQPNQVPVQPEATQVPLVSSTSEGYTASQPLYQPSHATEQRPQKEPIDQIQATISLNTDQTTASSSLPAASQPQVFQAGTSKPLHSSGINVNAAPFQSMQTVFNMNAPVPPVNEPETLKQQNQYQASYNQSFSSQPHQVEQTDLQQEQLQTVVGTYHGSQDQPHQVTGNHQQPPQQNTGFPRSSQPYYNSRGVSRGGSRGARGLMNGYRGPANGFRGGYDGYRPSFSNTPNSGYTQSQFSAPRDYSGYQRDGYQQNFKRGSGQSGPRGAPRGRGGPPRPNRGMPQMNTQQVN
atgccgtcggccaccagcctcagcggaagcggcagcaagtcgtcgggcccgccgcccccgtcgggttcctccgggagcgaggcggcggcggcggcgggggcggcgggggcggcgggggccggggcggctgcgcccgcctcccagcaccccgcgaccggcaccggcgctgtccagaccgaggccatgaagcagatcctcggggtgatcgacaagaaactccggaacctggagaagaaaaagggcaagcttgatgattaccaggaacgaatgaacaaaggggaaaggcttaatcaagatcagctggatgccgtatctaagtaccaggaagtcacaaataacttggagtttgcaaaagaattacagaggagtttcatggcattaagtcaagatattcagaaaacaataaagaagactgcacgtcgggagcagcttatgagagaggaagcggaacaaaaacgtttaaaaactgtacttgagctccagtatgttttggacaaattgggagatgatgaagtgagaactgacctgaagcaaggtttgaatggagtgccaatattgtctgaagaagaattgtcgttgttggatgaattctacaaattagcagaccctgaacgggacatgagcttgaggttgaatgagcagtatgaacatgcttccattcacctgtgggacttgctggaaggaaaggaaaagtctgtatgtggaacaacctataaagcactaaaggaaattgttgagcgtgttttccagtcaaattactttgacagcactcacaaccaccagaatgggctatgtgaggaagaagaggcagcctcagcacctacagttgaagaccaggtagctgaagctgagcctgagccagcagaagaatacactgaacaaagtgaagttgaatcaacagagtatgtaaatagacaatttatggcagaaacacagttcagcagtggtgaaaaggagcaggtagatgagtggacggtcgaaacagtggaggtggtgaattcactccagcagcaacctcaggctgcgtctccttcagtaccagagccccactctttgactccggtggctcaggcagatccccttgtgagaagacagcgagtccaggaccttatggcgcagatgcaggggccctataatttcatacaggattcaatgctggattttgaaaaccagacactcgatcctgccattgtatctgcacagcctatgaatccgacacaaaacatggacatgccccagctggtttgccctccagttcattctgaatctagacttgctcaacctaatcaagttcctgtacaaccagaagctacacaggttcctttggtttcatccacaagtgaggggtatacagcatctcaacccttgtaccagccttctcatgctacagagcaacgaccacaaaaggaaccaattgaccagattcaggcaacaatctctttaaatacagaccagactacagcgtcatcatcccttccggctgcttctcagcctcaggtattccaggctgggacaagcaaaccattacatagcagtggaatcaatgtaaatgcagctccattccaatccatgcaaacggtgttcaatatgaatgccccagttcctcctgttaatgaaccagaaactttgaaacaacaaaatcagtaccaggccagttataaccagagcttttctagtcagcctcaccaagtagaacaaacagaccttcagcaagaacagcttcaaacagtggttggcacttaccatggttcccaggaccagccccaccaagtgactggtaaccatcagcagcctccccagcagaacactggatttccacgtagcagtcagccctattacaatagtcgtggtgtgtctcgtggtggttcccgtggtgctagaggcttaatgaatggatacaggggccctgccaatggattcagaggaggatatgatggttaccgcccttcattctctaacactccaaacagtggttatacacagtctcagttcagtgctccccgggactactctggctatcagcgggatggatatcagcagaatttcaagcgaggctctgggcagagtggaccacggggagccccacgaggtcgtggagggcccccaagacccaacagagggatgccgcaaatgaacactcagcaagtgaattaatctgattcacaggattatgtttaaacgccaaaaacacactggccagtgtaccataatatgttaccagaagagttattatctatttgttctccctttcaggaaacttattgtaaagggactgttttcatcccataaagacaggactacaattgtcagctttatattacctggatatggaaggaaactatttttattctgcatgttcttcctaagcgtcatcttgagccttgcacatgatactcagattcctcacccttgcttaggagtaaaacataatacactttacagggtgatatctccatagttatttgaagtggcttggaaaaagcaagattaacttctgacattggataaaaatcaacaaatcagccctagagttattcaaatggtaattgacaaaaactaaaatatttcccttcgagaaggagtggaatgtggtttggcagaacaactgcatttcacagcttttccggttaaattggagcactaaacgtttagatgcataccaaattatgcatgggcccttaatataaaaggctggctaccagctttgacacagcactattcatcctctggccaaacaactgtggttaaacaacacatgtaaattgctttttaacagctgatactataataagacaaagccaaaatgcaaaaattgggctttgattggcactttttgaaaaatatgcaacaaatatgggatgtaatctggatggccgcttctgtacttaatgtgaagtatttagatacctttttgaacacttaacagtttcttctgacaatgacttttgtaaggattggtactatctatcattccttataatgtacattgtctgtcactaatcctcagatcttgctgtattgtcacctaaattggtacaggtactgatgaaaatatctaatggataatcataacactcttggtcacatgtttttcctgcagcctgaaggtttttaaaagaaaaagatatcaaatgcctgctgctaccacccttttaaattgctatcttttgaaaagcaccagtatgtgttttagattgatttccctattttagggaaatgacagacagtagtttcagttctgatggtataagcaaaacaaataaaacatgtttataaaagttgtatcttgaaacactggtgttcaacagctagcagcttatgtggttcaccccatgcattgttagtgtttcagattttatggttatctccagcagctgtttctgtagtacttgcatttatcttttgtctaaccctaatattctcacggaggcatttatattcaaagtggtgatcccttcacttagacgcatagggagagtcacaagtttgatgaagaggacagtgtagtaatttatatgctgttggaatttgtgctagcagtttgagcactagttctgtgtgcctatgaacttaatgctgcttgtcatattccactttgacttcatggagaattaatcccatctactcagcaaaggctatactaatactaagttaatggtattttctgtgcagaaattgaattttgttttattagcatttagctaaggaatttttccagtaggtgctcagctactaaagaaaaacaaaaacaagacacaaaactattctcaaacattcattgttagacaactggagtttttgctggttttgtaacctactaaaatggataggctgttgaacattccacattcaaaagttttttgtagggtggtggggaagggggggtgtcttcaatgtttattttaaaataaaataagttcttgacttttctcatgtgtggttgtggtacatcatattggaagggttatctgtttacttttgcaaatgagtatttctcttgctagcacctcccgttgtgcgctttaaatgacatctgcctgggatgtaccacaaccatatgttagctgtattttatggggaatagataaaatattcgtggtttattgggtaatccctagatgtgtatgcttacaatcctatatataaaactaaat

SEQ ID NO: 8 - protein, 717 aa, Canis familiaris
MPSATSLSGSGSKSSGPPPPSGSSGSEAAAAAGAAGAAGAGAAAPASQHPATGTGAVQTEAMKQILGVIDKKLRNLEKKKGKLDDYQERMNKGERLNQDQLDAVSKYQEVTNNLEFAKELQRSFMALSQDIQKTIKKTARREQLMREEAEQKRLKTVLELQYVLDKLGDDEVRTDLKQGLNGVPILSEEELSLLDEFYKLADPERDMSLRLNEQYEHASIHLWDLLEGKEKSVCGTTYKALKEIVERVFQSNYFDSTHNHQNGLCEEEEAASAPTVEDQVAEAEPEPAEEYTEQSEVESTEYVNRQFMAETQFSSGEKEQVDEWTVETVEVVNSLQQQPQAASPSVPEPHSLTPVAQADPLVRRQRVQDLMAQMQGPYNFIQDSMLDFENQTLDPAIVSAQPMNPTQNMDMPQLVCPPVHSESRLAQPNQVPVQPEATQVPLVSSTSEGYTASQPLYQPSHATEQRPQKEPIDQIQATISLNTDQTTASSSLPAASQPQVFQAGTSKPLHSSGINVNAAPFQSMQTVFNMNAPVPPVNEPETLKQQNQYQASYNQSFSSQPHQVEQTDLQQEQLQTVVGTYHGSQDQPHQVTGNHQQPPQQNTGFPRSSQPYYNSRGVSRGGSRGARGLMNGYRGPANGFRGGYDGYRPSFSNTPNSGYTQSQFSAPRDYSGYQRDGYQQNFKRGSGQSGPRGAPRGRGGPPRPNRGMPQMNTQQVN

SEQ ID NO: 9 - DNA, 4939 bp, Canis familiaris
  source 1..4939: mol_type = other DNA
  CDS 1..2109: protein_id = 314; translation = MPSATSLSGSGSKSSGPPPPSGSSGSEAAAAAGAAGAAGAGAAAPASQHPATGTGAVQTEAMKQILGVIDKKLRNLEKKKGKLDDYQERMNKGERLNQDQLDAVSKYQEVTNNLEFAKELQRSFMALSQDIQKTIKKTARREQLMREEAEQKRLKTVLELQYVLDKLGDDEVRTDLKQGLNGVPILSEEELSLLDEFYKLADPERDMSLRLNEQYEHASIHLWDLLEGKEKSVCGTTYKALKEIVERVFQSNYFDSTHNHQNGLCEEEEAASAPTVEDQVAEAEPEPAEEYTEQSEVESTEYVNRQFMAETQFSSGEKEQVDEWTVETVEVVNSLQQQPQAASPSVPEPHSLTPVAQADPLVRRQRVQDLMAQMQGPYNFIQDSMLDFENQTLDPAIVSAQPMNPTQNMDMPQLVCPPVHSESRLAQPNQVPVQPEATQVPLVSSTSEGYTASQPLYQPSHATEQRPQKEPIDQIQATISLNTDQTTASSSLPAASQPQVFQAGTSKPLHSSGINVNAAPFQSMQTVFNMNAPVPPVNEPETLKQQNQYQASYNQSFSSQPHQVEQTDLQQEQLQTVVGTYHGSQDQPHQVTGNHQQPPQQNTGFPRSSQPYYNSRGVSRGGSRGARGLMNGYRGPANGFRGGYDGYRPSFSNTPNSGYTQSQFSAPRDYSGYQRDGYQQNFKRGSGQSGPRGAPRGNILWW
atgccgtcggccaccagcctcagcggaagcggcagcaagtcgtcgggcccgccgcccccgtcgggttcctccgggagcgaggcggcggcggcggcgggggcggcgggggcggcgggggccggggcggctgcgcccgcctcccagcaccccgcgaccggcaccggcgctgtccagaccgaggccatgaagcagatcctcggggtgatcgacaagaaactccggaacctggagaagaaaaagggcaagcttgatgattaccaggaacgaatgaacaaaggggaaaggcttaatcaagatcagctggatgccgtatctaagtaccaggaagtcacaaataacttggagtttgcaaaagaattacagaggagtttcatggcattaagtcaagatattcagaaaacaataaagaagactgcacgtcgggagcagcttatgagagaggaagcggaacaaaaacgtttaaaaactgtacttgagctccagtatgttttggacaaattgggagatgatgaagtgagaactgacctgaagcaaggtttgaatggagtgccaatattgtctgaagaagaattgtcgttgttggatgaattctacaaattagcagaccctgaacgggacatgagcttgaggttgaatgagcagtatgaacatgcttccattcacctgtgggacttgctggaaggaaaggaaaagtctgtatgtggaacaacctataaagcactaaaggaaattgttgagcgtgttttccagtcaaattactttgacagcactcacaaccaccagaatgggctatgtgaggaagaagaggcagcctcagcacctacagttgaagaccaggtagctgaagctgagcctgagccagcagaagaatacactgaacaaagtgaagttgaatcaacagagtatgtaaatagacaatttatggcagaaacacagttcagcagtggtgaaaaggagcaggtagatgagtggacggtcgaaacagtggaggtggtgaattcactccagcagcaacctcaggctgcgtctccttcagtaccagagccccactctttgactccggtggctcaggcagatccccttgtgagaagacagcgagtccaggaccttatggcgcagatgcaggggccctataatttcatacaggattcaatgctggattttgaaaaccagacactcgatcctgccattgtatctgcacagcctatgaatccgacacaaaacatggacatgccccagctggtttgccctccagttcattctgaatctagacttgctcaacctaatcaagttcctgtacaaccagaagctacacaggttcctttggtttcatccacaagtgaggggtatacagcatctcaacccttgtaccagccttctcatgctacagagcaacgaccacaaaaggaaccaattgaccagattcaggcaacaatctctttaaatacagaccagactacagcgtcatcatcccttccggctgcttctcagcctcaggtattccaggctgggacaagcaaaccattacatagcagtggaatcaatgtaaatgcagctccattccaatccatgcaaacggtgttcaatatgaatgccccagttcctcctgttaatgaaccagaaactttgaaacaacaaaatcagtaccaggccagttataaccagagcttttctagtcagcctcaccaagtagaacaaacagaccttcagcaagaacagcttcaaacagtggttggcacttaccatggttcccaggaccagccccaccaagtgactggtaaccatcagcagcctccccagcagaacactggatttccacgtagcagtcagccctattacaatagtcgtggtgtgtctcgtggtggttcccgtggtgctagaggcttaatgaatggatacaggggccctgccaatggattcagaggaggatatgatggttaccgcccttcattctctaacactccaaacagtggttatacacagtctcagttcagtgctccccgggactactctggctatcagcgggatggatatcagcagaatttcaagcgaggctctgggcagagtggaccacggggagccccacgaggtaatattttgtggtggtgatcctagctcctaagtggagcttctgttctggccttggaagagctgttccatagtctgcatgtaggttacatgttaggaatacatttatcattaccagacttgttgctagggattaaatgaaatgctctgtttctaaaacttctcttgaacccaaatttaattttttgaatgactttccctgttactatataaattgtcttgaaaactagaacatttctcctcctcagaaaaagtgtttttccaactgcaaattatttttcaggtcctaaaacctgctaaatgtttttaggaagtacttactgaaacatttttgtaagacatttttggaatgagattgaacatttatataaatttattattattcctctttcatttttgaacatgcatattatattttagggtcagaaatcctttaatggccaaataagccatagttacatttagagaaccatttagaagtgatagaactaactgaaatttcaatgcctttggatcattaatagcgatataaatttcaaattgtttctgacttttaaataaaacatccaaaatcctaactaacttcctgaactatatttaaaaattacaggtttaaggagtttctggttttttttctcttaccataggaaaactgtttcctgtttggccaggaagtcaacctgtgtaataattagaagtagcatttcatatgatctgaagttctaaatggttctctgatttaagggaagttaaattgaataggtttcctctagttattggccataacatgtataaaatgtatattaaggaggaatacaaagtactttgatttcaatgctagtagaaactggccagcaaaaaggtgcattttatttttaaattaatggatcacttgggaattactgacttgaagtatcaaaggatatttgcatgtgaatgtgggttatgttctttctcaccttgtagcatattctatgaaagttgagttgactggtagctaaaaatctgttttaacagcatgtaaaaagttattttatctgttacaagtcattatacaattttgaatgttatgtagtttctttttaacagtttaggtaacaaggtctgtttttcattctggtgcttttattaattttgatagtatgatgttacttactactgaaatgtaagctagagtgtacactagaatgtaagctccatgagagcaggtaccttgtctgtcttcactgctgtatctatttccaacgcctgatgacagtgcctgacacatagtaggcactcaataaatacttgttgaatgaatgaatgaatgagtactggtggaatactccattagctctactcttcttttagctagagaacatgagcaaatttgcgcatgacaacttccaggacaggtgaacactgaagaattgacctcttaaacctaataatgtggtgacaagctgcccacatgcttcttgacttcagatgaaaatctgcttgaaggcaaagcaaataatatttgaaagaaaaaccaaatgccatttttgtcttctaggtcgtggagggcccccaagacccaacagagggatgccgcaaatgaacactcagcaagtgaattaatctgattcacaggattatgtttaaacgccaaaaacacactggccagtgtaccataatatgttaccagaagagttattatctatttgttctccctttcaggaaacttattgtaaagggactgttttcatcccataaagacaggactacaattgtcagctttatattacctggatatggaaggaaactatttttattctgcatgttcttcctaagcgtcatcttgagccttgcacatgatactcagattcctcacccttgcttaggagtaaaacataatacactttacagggtgatatctccatagttatttgaagtggcttggaaaaagcaagattaacttctgacattggataaaaatcaacaaatcagccctagagttattcaaatggtaattgacaaaaactaaaatatttcccttcgagaaggagtggaatgtggtttggcagaacaactgcatttcacagcttttccggttaaattggagcactaaacgtttagatgcataccaaattatgcatgggcccttaatataaaaggctggctaccagctttgacacagcactattcatcctctggccaaacaactgtggttaaacaacacatgtaaattgctttttaacagctgatactataataagacaaagccaaaatgcaaaaattgggctttgattggcactttttgaaaaatatgcaacaaatatgggatgtaatctggatggccgcttctgtacttaatgtgaagtatttagatacctttttgaacacttaacagtttcttctgacaatgacttttgtaaggattggtactatctatcattccttataatgtacattgtctgtcactaatcctcagatcttgctgtattgtcacctaaattggtacaggtactgatgaaaatatctaatggataatcataacactcttggtcacatgtttttcctgcagcctgaaggtttttaaaagaaaaagatatcaaatgcctgctgctaccacccttttaaattgctatcttttgaaaagcaccagtatgtgttttagattgatttccctattttagggaaatgacagacagtagtttcagttctgatggtataagcaaaacaaataaaacatgtttataaaagttgtatcttgaaacactggtgttcaacagctagcagcttatgtggttcaccccatgcattgttagtgtttcagattttatggttatctccagcagctgtttctgtagtacttgcatttatc

SEQ ID NO: 10 - protein, 702 aa, Canis familiaris
MPSATSLSGSGSKSSGPPPPSGSSGSEAAAAAGAAGAAGAGAAAPASQHPATGTGAVQTEAMKQILGVIDKKLRNLEKKKGKLDDYQERMNKGERLNQDQLDAVSKYQEVTNNLEFAKELQRSFMALSQDIQKTIKKTARREQLMREEAEQKRLKTVLELQYVLDKLGDDEVRTDLKQGLNGVPILSEEELSLLDEFYKLADPERDMSLRLNEQYEHASIHLWDLLEGKEKSVCGTTYKALKEIVERVFQSNYFDSTHNHQNGLCEEEEAASAPTVEDQVAEAEPEPAEEYTEQSEVESTEYVNRQFMAETQFSSGEKEQVDEWTVETVEVVNSLQQQPQAASPSVPEPHSLTPVAQADPLVRRQRVQDLMAQMQGPYNFIQDSMLDFENQTLDPAIVSAQPMNPTQNMDMPQLVCPPVHSESRLAQPNQVPVQPEATQVPLVSSTSEGYTASQPLYQPSHATEQRPQKEPIDQIQATISLNTDQTTASSSLPAASQPQVFQAGTSKPLHSSGINVNAAPFQSMQTVFNMNAPVPPVNEPETLKQQNQYQASYNQSFSSQPHQVEQTDLQQEQLQTVVGTYHGSQDQPHQVTGNHQQPPQQNTGFPRSSQPYYNSRGVSRGGSRGARGLMNGYRGPANGFRGGYDGYRPSFSNTPNSGYTQSQFSAPRDYSGYQRDGYQQNFKRGSGQSGPRGAPRGNILWW

SEQ ID NO: 11 - DNA, 3306 bp, Canis familiaris
  source 1..3306: mol_type = other DNA
  CDS 1..2040: protein_id = 315; translation = MPSATSLSGSGSKSSGPPPPSGSSGSEAAAAAGAAGAAGAGAAAPASQHPATGTGAVQTEAMKQILGVIDKKLRNLEKKKGKLDDYQERMNKGERLNQDQLDAVSKYQEVTNNLEFAKELQRSFMALSQDIQKTIKKTARREQLMREEAEQKRLKTVLELQYVLDKLGDDEVRTDLKQGLNGVPILSEEELSLLDEFYKLADPERDMSLRLNEQYEHASIHLWDLLEGKEKSVCGTTYKALKEIVERVFQSNYFDSTHNHQNGLCEEEEAASAPTVEDQVAEAEPEPAEEYTEQSEVESTEYVNRQFMAETQFSSGEKEQVDEWTVETVEVVNSLQQQPQAASPSVPEPHSLTPVAQADPLVRRQRVQDLMAQMQGPYNFIQDSMLDFENQTLDPAIVSAQPMNPTQNMDMPQLVCPPVHSESRLAQPNQVPVQPEATQVPLVSSTSEGYTASQPLYQPSHATEQRPQKEPIDQIQATISLNTDQTTASSSLPAASQPQVFQAGTSKPLHSSGINVNAAPFQSMQTVFNMNAPVPPVNEPETLKQQNQYQASYNQSFSSQPHQVEQTDLQQEQLQTVVGTYHGSQDQPHQVTGNHQQPPQQNTGFPRSSQPYYNSRGVSRGGSRGARGLMNGYRGPANGFRGGYDGYRPSFSNTPNSGYTQSQFSAPRDYSGYQRGCRK
atgccgtcggccaccagcctcagcggaagcggcagcaagtcgtcgggcccgccgcccccgtcgggttcctccgggagcgaggcggcggcggcggcgggggcggcgggggcggcgggggccggggcggctgcgcccgcctcccagcaccccgcgaccggcaccggcgctgtccagaccgaggccatgaagcagatcctcggggtgatcgacaagaaactccggaacctggagaagaaaaagggcaagcttgatgattaccaggaacgaatgaacaaaggggaaaggcttaatcaagatcagctggatgccgtatctaagtaccaggaagtcacaaataacttggagtttgcaaaagaattacagaggagtttcatggcattaagtcaagatattcagaaaacaataaagaagactgcacgtcgggagcagcttatgagagaggaagcggaacaaaaacgtttaaaaactgtacttgagctccagtatgttttggacaaattgggagatgatgaagtgagaactgacctgaagcaaggtttgaatggagtgccaatattgtctgaagaagaattgtcgttgttggatgaattctacaaattagcagaccctgaacgggacatgagcttgaggttgaatgagcagtatgaacatgcttccattcacctgtgggacttgctggaaggaaaggaaaagtctgtatgtggaacaacctataaagcactaaaggaaattgttgagcgtgttttccagtcaaattactttgacagcactcacaaccaccagaatgggctatgtgaggaagaagaggcagcctcagcacctacagttgaagaccaggtagctgaagctgagcctgagccagcagaagaatacactgaacaaagtgaagttgaatcaacagagtatgtaaatagacaatttatggcagaaacacagttcagcagtggtgaaaaggagcaggtagatgagtggacggtcgaaacagtggaggtggtgaattcactccagcagcaacctcaggctgcgtctccttcagtaccagagccccactctttgactccggtggctcaggcagatccccttgtgagaagacagcgagtccaggaccttatggcgcagatgcaggggccctataatttcatacaggattcaatgctggattttgaaaaccagacactcgatcctgccattgtatctgcacagcctatgaatccgacacaaaacatggacatgccccagctggtttgccctccagttcattctgaatctagacttgctcaacctaatcaagttcctgtacaaccagaagctacacaggttcctttggtttcatccacaagtgaggggtatacagcatctcaacccttgtaccagccttctcatgctacagagcaacgaccacaaaaggaaccaattgaccagattcaggcaacaatctctttaaatacagaccagactacagcgtcatcatcccttccggctgcttctcagcctcaggtattccaggctgggacaagcaaaccattacatagcagtggaatcaatgtaaatgcagctccattccaatccatgcaaacggtgttcaatatgaatgccccagttcctcctgttaatgaaccagaaactttgaaacaacaaaatcagtaccaggccagttataaccagagcttttctagtcagcctcaccaagtagaacaaacagaccttcagcaagaacagcttcaaacagtggttggcacttaccatggttcccaggaccagccccaccaagtgactggtaaccatcagcagcctccccagcagaacactggatttccacgtagcagtcagccctattacaatagtcgtggtgtgtctcgtggtggttcccgtggtgctagaggcttaatgaatggatacaggggccctgccaatggattcagaggaggatatgatggttaccgcccttcattctctaacactccaaacagtggttatacacagtctcagttcagtgctccccgggactactctggctatcagcggggatgccgcaaatgaacactcagcaagtgaattaatctgattcacaggattatgtttaaacgccaaaaacacactggccagtgtaccataatatgttaccagaagagttattatctatttgttctccctttcaggaaacttattgtaaagggactgttttcatcccataaagacaggactacaattgtcagctttatattacctggatatggaaggaaactatttttattctgcatgttcttcctaagcgtcatcttgagccttgcacatgatactcagattcctcacccttgcttaggagtaaaacataatacactttacagggtgatatctccatagttatttgaagtggcttggaaaaagcaagattaacttctgacattggataaaaatcaacaaatcagccctagagttattcaaatggtaattgacaaaaactaaaatatttcccttcgagaaggagtggaatgtggtttggcagaacaactgcatttcacagcttttccggttaaattggagcactaaacgtttagatgcataccaaattatgcatgggcccttaatataaaaggctggctaccagctttgacacagcactattcatcctctggccaaacaactgtggttaaacaacacatgtaaattgctttttaacagctgatactataataagacaaagccaaaatgcaaaaattgggctttgattggcactttttgaaaaatatgcaacaaatatgggatgtaatctggatggccgcttctgtacttaatgtgaagtatttagatacctttttgaacacttaacagtttcttctgacaatgacttttgtaaggattggtactatctatcattccttataatgtacattgtctgtcactaatcctcagatcttgctgtattgtcacctaaattggtacaggtactgatgaaaatatctaatggataatcataacactcttggtcacatgtttttcctgcagcctgaaggtttttaaaagaaaaagatatcaaatgcctgctgctaccacccttttaaattgctatcttttgaaaagcaccagtatgtgttttagattgatttccctattttagggaaatgacagacagtagtttcagttctgatggtataagcaaaacaaataaaacatgtttataaaagttgtatcttgaaacactggtgttcaacagctagcagcttatgtggttcaccccatgcattgttagtgtttcagattttatggttatctccagcagctgtttctgtagtacttgcatttatc

SEQ ID NO: 12 - protein, 679 aa, Canis familiaris
MPSATSLSGSGSKSSGPPPPSGSSGSEAAAAAGAAGAAGAGAAAPASQHPATGTGAVQTEAMKQILGVIDKKLRNLEKKKGKLDDYQERMNKGERLNQDQLDAVSKYQEVTNNLEFAKELQRSFMALSQDIQKTIKKTARREQLMREEAEQKRLKTVLELQYVLDKLGDDEVRTDLKQGLNGVPILSEEELSLLDEFYKLADPERDMSLRLNEQYEHASIHLWDLLEGKEKSVCGTTYKALKEIVERVFQSNYFDSTHNHQNGLCEEEEAASAPTVEDQVAEAEPEPAEEYTEQSEVESTEYVNRQFMAETQFSSGEKEQVDEWTVETVEVVNSLQQQPQAASPSVPEPHSLTPVAQADPLVRRQRVQDLMAQMQGPYNFIQDSMLDFENQTLDPAIVSAQPMNPTQNMDMPQLVCPPVHSESRLAQPNQVPVQPEATQVPLVSSTSEGYTASQPLYQPSHATEQRPQKEPIDQIQATISLNTDQTTASSSLPAASQPQVFQAGTSKPLHSSGINVNAAPFQSMQTVFNMNAPVPPVNEPETLKQQNQYQASYNQSFSSQPHQVEQTDLQQEQLQTVVGTYHGSQDQPHQVTGNHQQPPQQNTGFPRSSQPYYNSRGVSRGGSRGARGLMNGYRGPANGFRGGYDGYRPSFSNTPNSGYTQSQFSAPRDYSGYQRGCRK

SEQ ID NO: 13 - DNA, 2281 bp, Canis familiaris
  source 1..2281: mol_type = other DNA
  CDS 1..2154: protein_id = 316; translation = MPSATSLSGSGSKSSGPPPPSGSSGSEAAAAAGAAGAAGAGAAAPASQHPATGTGAVQTEAMKQILGVIDKKLRNLEKKKGKLDDYQERMNKGERLNQDQLDAVSKYQEVTNNLEFAKELQRSFMALSQDIQKTIKKTARREQLMREEAEQKRLKTVLELQYVLDKLGDDEVRTDLKQGLNGVPILSEEELSLLDEFYKLADPERDMSLRLNEQYEHASIHLWDLLEGKEKSVCGTTYKALKEIVERVFQSNYFDSTHNHQNGLCEEEEAASAPTVEDQVAEAEPEPAEEYTEQSEVESTEYVNRQFMAETQFSSGEKEQVDEWTVETVEVVNSLQQQPQAASPSVPEPHSLTPVAQADPLVRRQRVQDLMAQMQGPYNFIQDSMLDFENQTLDPAIVSAQPMNPTQNMDMPQLVCPPVHSESRLAQPNQVPVQPEATQVPLVSSTSEGYTASQPLYQPSHATEQRPQKEPIDQIQATISLNTDQTTASSSLPAASQPQVFQAGTSKPLHSSGINVNAAPFQSMQTVFNMNAPVPPVNEPETLKQQNQYQASYNQSFSSQPHQVEQTDLQQEQLQTVVGTYHGSQDQPHQVTGNHQQPPQQNTGFPRSSQPYYNSRGVSRGGSRGARGLMNGYRGPANGFRGGYDGYRPSFSNTPNSGYTQSQFSAPRDYSGYQRDGYQQNFKRGSGQSGPRGAPRGRGGPPRPNRGMPQMNTQQVN
atgccgtcggccaccagcctcagcggaagcggcagcaagtcgtcgggcccgccgcccccgtcgggttcctccgggagcgaggcggcggcggcggcgggggcggcgggggcggcgggggccggggcggctgcgcccgcctcccagcaccccgcgaccggcaccggcgctgtccagaccgaggccatgaagcagatcctcggggtgatcgacaagaaactccggaacctggagaagaaaaagggcaagcttgatgattaccaggaacgaatgaacaaaggggaaaggcttaatcaagatcagctggatgccgtatctaagtaccaggaagtcacaaataacttggagtttgcaaaagaattacagaggagtttcatggcattaagtcaagatattcagaaaacaataaagaagactgcacgtcgggagcagcttatgagagaggaagcggaacaaaaacgtttaaaaactgtacttgagctccagtatgttttggacaaattgggagatgatgaagtgagaactgacctgaagcaaggtttgaatggagtgccaatattgtctgaagaagaattgtcgttgttggatgaattctacaaattagcagaccctgaacgggacatgagcttgaggttgaatgagcagtatgaacatgcttccattcacctgtgggacttgctggaaggaaaggaaaagtctgtatgtggaacaacctataaagcactaaaggaaattgttgagcgtgttttccagtcaaattactttgacagcactcacaaccaccagaatgggctatgtgaggaagaagaggcagcctcagcacctacagttgaagaccaggtagctgaagctgagcctgagccagcagaagaatacactgaacaaagtgaagttgaatcaacagagtatgtaaatagacaatttatggcagaaacacagttcagcagtggtgaaaaggagcaggtagatgagtggacggtcgaaacagtggaggtggtgaattcactccagcagcaacctcaggctgcgtctccttcagtaccagagccccactctttgactccggtggctcaggcagatccccttgtgagaagacagcgagtccaggaccttatggcgcagatgcaggggccctataatttcatacaggattcaatgctggattttgaaaaccagacactcgatcctgccattgtatctgcacagcctatgaatccgacacaaaacatggacatgccccagctggtttgccctccagttcattctgaatctagacttgctcaacctaatcaagttcctgtacaaccagaagctacacaggttcctttggtttcatccacaagtgaggggtatacagcatctcaacccttgtaccagccttctcatgctacagagcaacgaccacaaaaggaaccaattgaccagattcaggcaacaatctctttaaatacagaccagactacagcgtcatcatcccttccggctgcttctcagcctcaggtattccaggctgggacaagcaaaccattacatagcagtggaatcaatgtaaatgcagctccattccaatccatgcaaacggtgttcaatatgaatgccccagttcctcctgttaatgaaccagaaactttgaaacaacaaaatcagtaccaggccagttataaccagagcttttctagtcagcctcaccaagtagaacaaacagaccttcagcaagaacagcttcaaacagtggttggcacttaccatggttcccaggaccagccccaccaagtgactggtaaccatcagcagcctccccagcagaacactggatttccacgtagcagtcagccctattacaatagtcgtggtgtgtctcgtggtggttcccgtggtgctagaggcttaatgaatggatacaggggccctgccaatggattcagaggaggatatgatggttaccgcccttcattctctaacactccaaacagtggttatacacagtctcagttcagtgctccccgggactactctggctatcagcgggatggatatcagcagaatttcaagcgaggctctgggcagagtggaccacggggagccccacgaggtcgtggagggcccccaagacccaacagagggatgccgcaaatgaacactcagcaagtgaattaatctgattcacaggattatgtttaaacgccaaaaacacactggccagtgtaccataatatgttaccagaagagttattatctatttggactgttttcatcccataaagacaggactacaattgtcagc

SEQ ID NO: 14 - protein, 717 aa, Canis familiaris; identical to SEQ ID NO: 8

SEQ ID NO: 15 - DNA, 3386 bp, Bos taurus
  source 1..3386: mol_type = other DNA
  CDS 82..2208: protein_id = 317; translation = MPSATSHSGSGSKSSGPPPPSGSSGNEAGAGAAAPASQHPMTGTGAVQTEAMKQILGVIDKKLRNLEKKKGKLDDYQERMNKGERLNQDQLDAVSKYQEVTNNLEFAKELQRSFMALSQDIQKTIKKTARREQLMREEAEQKRLKTVLELQYVLDKLGDDEVRTDLKQGLNGVPILSEEELSLLDEFYKLADPERDMSLRLNEQYEHASIHLWDLLEGKEKPVCGTTYKALKEIVERVFQSNYFDSTHNHQNGLCEEEEAASAPTVEDQAAEAEPEPVEEYTEQNEVESTEYVNRQFMAETQFSSGEKEQVDDWTVETVEVVNSLQQQPQAASPSVPEPHSLTPVAQADPLVRRQRVQDLMAQMQGPYNFIQDSMLDFENQTLDPAIVSAQPMNPAQNMDIPQLVCPPVHSESRLAQPNQVSVQPEATQVPLVSSTSEGYTASQPLYQPSHATDQRPQKEPIDQIQATISLNTDQTTASSSLPAASQPQVFQAGTSKPLHSSGINVNAAPFQSMQTVFNMNAPVPPVNEPETLKQQNQYQASYNQSFSSQPHQVEQTELQQEQLQTVVGTYHGSQDQPHQVTGNHQQPPQQNTGFPRSNQPYYNSRGVSRGGSRGARGLMNGYRGPANGFRGGYDGYRPSFSTNTPNSGYTQSQFSAPRDYSGYQRDGYQQNFKRGSGQSGPRGAPRGRGGPPRPNRGMPQMNTQQVN
cgcgtctcgccccgtccaccgattgactcgccgctcttgtccttcctcccgctctttcttctctccccttacggtttcaagatgccttcggccaccagccacagcggaagcggcagcaagtcgtccggaccgccaccgccgtcgggttcctccgggaatgaggcgggggccggggccgccgcgccggcttcccaacaccccatgaccggcaccggggctgtccagaccgaggccatgaagcagattctcggggtgatcgacaagaaacttcggaacctggagaagaaaaagggcaagcttgatgattatcaggaacgaatgaacaaaggggaaaggcttaatcaagatcagctggatgccgtgtctaagtaccaggaagtcacaaataacttggagtttgcaaaagaattacagaggagtttcatggcattaagccaagatattcagaaaacaataaagaagacagcacgtcgggagcagcttatgagagaggaagctgaacagaaacgtttaaaaacagtacttgagctgcagtatgttttggacaaactaggagatgatgaagtgagaactgacctgaagcaaggtttgaatggagtgccaatattgtctgaagaggagttgtcgttgttagatgagttctacaaattagcagaccctgaacgagacatgagcttgaggttgaatgagcagtatgaacatgcctccattcacctgtgggacttgctggaaggaaaggaaaaacctgtatgtggaacaacttataaagctctaaaggaaattgttgagcgtgttttccagtcaaactactttgacagcacccacaaccaccagaatggtctgtgtgaggaagaggaggcagcctcagcacctacagttgaagaccaggcagctgaagctgaacctgagccagtggaagaatatactgaacaaaatgaggttgaatcaacagagtatgtaaatagacaatttatggcagaaacacagttcagcagtggtgaaaaggagcaggtagatgattggacagttgaaacagttgaggtggtaaattcactccagcagcaacctcaggctgcatctccttcagtaccagaaccccactctttgaccccagtggctcaagccgatcccctcgtgagaagacagcgagtacaggaccttatggcacaaatgcaggggccctataatttcatacaggattcaatgttggattttgaaaaccagacacttgatcctgccattgtatctgcacagccgatgaatccagcacagaacatggacataccccagctggtttgccctccagttcattctgaatctagacttgctcaacctaatcaagtttctgtacagccagaagctacacaggttcctttggtttcatccacaagtgagggatatacagcatctcaacccttgtaccaaccttctcatgctactgaccaacgaccacaaaaggaaccgattgatcagattcaggcgacgatctctttaaatacagaccagactacagcatcatcatcccttcctgctgcttctcagcctcaagtgttccaggctgggacaagcaaacctttacatagcagtggaatcaatgtaaatgcagctccattccaatccatgcaaacggtattcaatatgaatgccccagttcctcctgttaatgaaccagaaactttaaaacagcaaaatcagtaccaggccagttacaaccagagcttttccagtcagcctcaccaagtagaacaaacagagcttcagcaagaacagcttcaaacagtggttggcacttatcatggttctcaggaccagccccatcaagtgactggtaaccaccagcagcctcctcagcagaacactggatttccacgtagcaatcagccctattacaacagtcgtggtgtgtctcgtggaggttcccgtggtgctagaggcttgatgaatggatacagaggacctgctaatggattcagaggaggatatgatggttaccgcccttcattctctactaacactccaaacagtggttatacacaatctcaattcagtgctccccgggactactctggctatcagcgggatggatatcagcagaatttcaagcgaggctctgggcagagtggaccacggggagccccacgaggtcgtggagggcccccaagacccaacagagggatgccgcaaatgaacactcagcaagtgaattaatctgattcacaggattatgtttaatcgccaaaaacacactggccagtgtaccataatatgttaccagaagagttattatctatttgttctccctttcaggaaacttattgtaaagggactgttttcatcccataaagacaggactacaattgtcagctttatattacctggatatggaaggaaactatttttactctgcatgttctgtcctaagcgtcatcttgagccttgcacatgatactcagattcctcacccttgcttaggagtaaaacataatatactttaatggggtgatatctccatagttatttgaagtggcttggataaagcaagactgacttctgacattggataaaatctacaaatcagccctagagtcattcagtggtaactgacaaaactaaaatatttcccttgaaaggaagatggaaggagtggagtgtggtttggcagaacaactgcatttcacagcttttccacttaaattggagcactgaacatttagatgcataccgaattatgcatgggccctaatcacacagacaaggctggtgccagccttaggcttgacacggcagtgttcaccctctggccagacgactgtggttcaagacacatgtaaattgctttttaacagctgatactgtataagacaaagccaaaatgcaaaattaggctttgattggcacttttcgaaaaatatgcaacaattaagggatataatctggatggccgcttctgtacttaatgtgaaatatttagatacctttcaaacacttaacagtttctttgacaatgagttttgtaaggattggtagtaaatatcattccttatgacgtacattgtctgtcactaatccttggatcttgctgtattgtcacctaaattggtacaggtactgatgaaaatctaatggataatcataacactcttggttacatgtttttcctgcagcctgaaagtttttataagaaaaagacatcaaatgcctgctgctgccacccttttaaattgctatcttttgaaaagcaccagtatgtgttttagattgatttccctattttagggaaatgacagtcagtagtttcacttctgatggtataagcaaacaaataaaacatgtttataaaaaaaaaaaaaaaaaaaaaaaaaaaaaaaaaaaaaaaaaaaaaaaaa

SEQ ID NO: 16 - protein, 708 aa, Bos taurus
MPSATSHSGSGSKSSGPPPPSGSSGNEAGAGAAAPASQHPMTGTGAVQTEAMKQILGVIDKKLRNLEKKKGKLDDYQERMNKGERLNQDQLDAVSKYQEVTNNLEFAKELQRSFMALSQDIQKTIKKTARREQLMREEAEQKRLKTVLELQYVLDKLGDDEVRTDLKQGLNGVPILSEEELSLLDEFYKLADPERDMSLRLNEQYEHASIHLWDLLEGKEKPVCGTTYKALKEIVERVFQSNYFDSTHNHQNGLCEEEEAASAPTVEDQAAEAEPEPVEEYTEQNEVESTEYVNRQFMAETQFSSGEKEQVDDWTVETVEVVNSLQQQPQAASPSVPEPHSLTPVAQADPLVRRQRVQDLMAQMQGPYNFIQDSMLDFENQTLDPAIVSAQPMNPAQNMDIPQLVCPPVHSESRLAQPNQVSVQPEATQVPLVSSTSEGYTASQPLYQPSHATDQRPQKEPIDQIQATISLNTDQTTASSSLPAASQPQVFQAGTSKPLHSSGINVNAAPFQSMQTVFNMNAPVPPVNEPETLKQQNQYQASYNQSFSSQPHQVEQTELQQEQLQTVVGTYHGSQDQPHQVTGNHQQPPQQNTGFPRSNQPYYNSRGVSRGGSRGARGLMNGYRGPANGFRGGYDGYRPSFSTNTPNSGYTQSQFSAPRDYSGYQRDGYQQNFKRGSGQSGPRGAPRGRGGPPRPNRGMPQMNTQQVN

SEQ ID NO: 17 - DNA, 3150 bp, Equus caballus
  source 1..3150: mol_type = other DNA
  CDS 1..1917: protein_id = 318; translation = MEGKLDDYQERMNKGERLNQDQLDAVSKYQEVTNNLEFAKELQRSFMALSQDIQKTIKKTARREQLMREEAEQKRLKTVLELQYVLDKLGDEEVRTDLKQGLNGVPILSEEELSLLDEFYKLADPVRDMSLRLNEQYEHASIHLWDLLEGKEKSVCGTTYKALREIVERVFQSNYFDSTHNHQNGLCEEEEATSAPTAEDQGAEAEPEPAEEYTEQSEVESTEYVNRQFMAEAQFSGEKEQVDEWTVETVEVVNSLQQQPQAASPSVPEPHSLTPVAQADPLVRRQRVQDLMAQMQGPYNFIQDSMLDFENQTLDPAIVSAQPMNPAQNMDMPQLVCPPVHAESRLAQPNQVPVQPEATQVPLVSSTSEGYTASQPLYQPSHATEQRPQKEPTDQIQATISLNTDQTTASSSLPAASQPQVFQAGTSKPLHSSGINVNAAPFQSMQTVFNMNAPVPPVNEPETLKQQNQYQASYNQSFSSPPHQVEQTELPQEQLQTVVGTYHASQDQPHQVTGNHQQPPQQNTGFPRSSQPYYNSRGVSRGGSRGARGLMNGYRGPANGFRGGYDGYRPSFSNTPNSGYTQSQFSAPRDYSGYQRDGYQQNFKRGSGQSGPRGAPRGRGGPPRPNRGMPQMNTQQVN
atggagggcaagctcgatgattaccaagagcgaatgaacaaaggagaaaggcttaatcaggatcagctggatgctgtgtctaagtaccaggaagtcacaaataacttggagtttgcgaaagaattgcagaggagtttcatggcgttgagtcaggatattcagaaaacaataaagaagacggcacgtcgggagcagcttatgagagaagaagctgaacagaaacgtttaaaaactgtacttgagctgcagtatgttttggacaaattgggagatgaagaagtgcgaactgacctgaaacaaggtttgaatggagtgccaatactctctgaagaagagttgtcgctgttggatgagttctacaagttagcagaccctgtacgggacatgagcttgaggttgaatgagcagtatgagcatgcctccattcacctgtgggacttgctggaagggaaggaaaaatctgtctgtggaacaacctataaagctctgagggaaattgttgagcgtgttttccagtccaactactttgacagcacccacaaccaccagaatgggctctgtgaggaggaagaggctacctcagctccaacagctgaagaccagggagctgaagctgaacctgagccagcagaagaatacactgaacaaagtgaagttgaatcaacagagtatgtaaatagacagtttatggcagaagcgcagttcagtggtgagaaggagcaggtggatgagtggacagtcgagacggtcgaggtggtaaattcactccagcagcaacctcaggctgcatctccttcagtaccggagccccactctttgactccagtggctcaggcagatccccttgtgagaagacagcgagtacaggaccttatggcgcaaatgcaggggccctataatttcatacaggattcaatgctggattttgaaaaccagacacttgatcctgccattgtatctgcacagcctatgaatccagcacagaatatggacatgccccagctggtttgccctccagttcatgctgaatctagacttgctcaacctaatcaagttcctgtacaaccagaagctacacaggttcctttggtttcatccacaagtgaggggtatacagcatctcagcccttgtaccagccttctcatgctacagagcaacgaccgcaaaaggaaccgactgaccagatccaggcaacaatctctttaaatacagaccagactacagcatcatcatcccttcctgctgcttctcagcctcaggtgttccaggctgggacaagcaaacctttacacagcagtgggatcaatgtaaatgcagcgccattccagtccatgcaaacggtgttcaacatgaatgccccggttcctcctgttaatgaaccagaaactttaaaacagcaaaatcagtaccaggccagctataaccagagcttttccagtccgcctcaccaagtagagcagacagagcttccgcaagagcagcttcagacggtggttggtacttaccatgcttcccaagaccagccccatcaagtgaccggtaaccaccagcagcctccccagcagaacactgggtttccacgtagcagtcagccctattacaacagtcgtggtgtgtctcgtggaggctcccgtggtgctagaggcttgatgaatggatacaggggccctgccaatggattcagaggaggatatgatggttaccgcccttcgttctctaacactccaaacagcggttacacacagtctcagttcagtgctccccgggactactctggctatcagcgggatggatatcagcagaatttcaagcgaggctctgggcagagtggaccccggggagccccacgaggtcgtggagggcccccaagacccaacagagggatgccgcaaatgaacactcagcaagtgaattaatctgattcacaggattatctttaatcgccaaaacacactggccagtgtaccataatatgttaccagaagagttattatctatttgttctccctttcaggaaacttattgtaaagggactgttttcatcccataaagacaggactacagttgtcagctttatattacctggatatggaaggaaactatttttactctgcatgttctgtcctaagcgtcatcttgagccttgcacatgatactcagattcctttcccttgcttaggagtaaaacataatatactttatggggtgataatatctccatagttatttgaagtggcttggaaaaagcaagattgacttttgacattggataaaatctacaaatcagccctagagtttcatggtcattcacaaaactaaaatatttcccttgaaaggaagatggaaggactggagtgtggtttggcagaacaactgcatttcacagcttttcctattaaattggagcactgaatgttaaatgcataccaaattatgcatgggcccttaatcacacatacatggctaccagctttgacacagcactattcatcctctggccaaacgactgtggttaaaaacacgtgtaaattgctttttaacagctgatactgtaaaagacaaagctaaaatgcaaaattaggctttcattggcacttttcgaaaaatatgcaacaaatttgggatgtaatctggatggccacttctgtacttaatgtgaagtatttagatacctttttgaacacttaacagtttcttcgacaatgacttttgtaaggattggtagtatatatcattccttatgacatacattgtctgttgctaatccttggatcttgctgtattgtcacctaaattggtacaggtactgatgaaaatctctcatggataaacctaacactcttcgtcacatgtttttcctgcagcctgaaggtttttaaaaggaaaagatatcaaatgcctgctgctaccacccttttaaattgctatcttttgaaaagcaccagtatgtgtttttagattgatttccctattttagggaaatgacagtcagtagtttcagttctgatggtataagcaaagcaaataaaacgtgtttataaaagttgtatcttgaaacactggtgttcaacagctagcagcttctgtggttcaccccctgccttgttagtgttacccatttatggttatctccagcagcaatttctcta

SEQ ID NO: 18 - protein, 638 aa, Equus caballus
MEGKLDDYQERMNKGERLNQDQLDAVSKYQEVTNNLEFAKELQRSFMALSQDIQKTIKKTARREQLMREEAEQKRLKTVLELQYVLDKLGDEEVRTDLKQGLNGVPILSEEELSLLDEFYKLADPVRDMSLRLNEQYEHASIHLWDLLEGKEKSVCGTTYKALREIVERVFQSNYFDSTHNHQNGLCEEEEATSAPTAEDQGAEAEPEPAEEYTEQSEVESTEYVNRQFMAEAQFSGEKEQVDEWTVETVEVVNSLQQQPQAASPSVPEPHSLTPVAQADPLVRRQRVQDLMAQMQGPYNFIQDSMLDFENQTLDPAIVSAQPMNPAQNMDMPQLVCPPVHAESRLAQPNQVPVQPEATQVPLVSSTSEGYTASQPLYQPSHATEQRPQKEPTDQIQATISLNTDQTTASSSLPAASQPQVFQAGTSKPLHSSGINVNAAPFQSMQTVFNMNAPVPPVNEPETLKQQNQYQASYNQSFSSPPHQVEQTELPQEQLQTVVGTYHASQDQPHQVTGNHQQPPQQNTGFPRSSQPYYNSRGVSRGGSRGARGLMNGYRGPANGFRGGYDGYRPSFSNTPNSGYTQSQFSAPRDYSGYQRDGYQQNFKRGSGQSGPRGAPRGRGGPPRPNRGMPQMNTQQVN

SEQ ID NO: 19 - DNA, 6181 bp, Mus musculus
  source 1..6181: mol_type = other DNA
  CDS 179..2302: protein_id = 319; translation = MPSATSHSGSGSKSSGPPPPSGSSGSEAAAGAAAPASQHPATGTGAVQTEAMKQILGVIDKKLRNLEKKKGKLDDYQERMNKGERLNQDQLDAVSKYQEVTNNLEFAKELQRSFMALSQDIQKTIKKTARREQLMREEAEQKRLKTVLELQYVLDKLGDDDVRTDLKQGLSGVPILSEEELSLLDEFYKLVDPERDMSLRLNEQYEHASIHLWDLLEGKEKPVCGTTYKALKEIVERVFQSNYFDSTHNHQNGLCEEEEAASAPTVEDQVAEAEPEPAEEYTEQSEVESTEYVNRQFMAETQFSSGEKEQVDEWTVETVEVVNSLQQQPQAASPSVPEPHSLTPVAQSDPLVRRQRVQDLMAQMQGPYNFIQDSMLDFENQTLDPAIVSAQPMNPTQNMDMPQLVCPQVHSESRLAQSNQVPVQPEATQVPLVSSTSEGYTASQPLYQPSHATEQRPQKEPMDQIQATISLNTDQTTASSSLPAASQPQVFQAGTSKPLHSSGINVNAAPFQSMQTVFNMNAPVPPANEPETLKQQSQYQATYNQSFSSQPHQVEQTELQQDQLQTVVGTYHGSQDQPHQVPGNHQQPPQQNTGFPRSSQPYYNSRGVSRGGSRGARGLMNGYRGPANGFRGGYDGYRPSFSNTPNSGYSQSQFTAPRDYSGYQRDGYQQNFKRGSGQSGPRGAPRGRGGPPRPNRGMPQMNTQQVN
gctggctggctaagtccctcccgcgccggctcttgtcccactaggagcagctcagagccgcggggacagggcgaagcggcctgcgcccacggagcgcacgtctctgttctcaacgcagcaccacccttgcccccctcggctgcccactccagacgtccagcggctccgcgcgcgcacgatgccctcggccaccagccacagcggaagcggcagcaaatcgtcgggaccgccgccgccgtccggttcctccgggagtgaggcggcggccggggcagctgcgccggcttctcagcatccggcaaccggcaccggcgccgtccagaccgaggccatgaagcagattctcggcgtaatcgacaagaaacttcggaacctggagaagaaaaagggtaaacttgatgattaccaggaacgaatgaataaaggggaaaggctcaatcaagaccagctggatgccgtatctaagtaccaggaagtcacaaataatttggagtttgcaaaggaattacagaggagtttcatggcattaagtcaagatattcagaaaacaataaagaagacagcacgtcgggaacagcttatgagagaagaagcagaacagaagcgcttaaaaactgtacttgagttacagtatgtattggataagctgggagatgatgatgtgagaacagatctgaaacaaggtttgagtggagtgccaatattgtctgaggaggagttgtcattgctggatgagttctacaagctcgtagatcctgagcgtgacatgagtttaaggttaaatgagcagtatgaacatgcctcaattcacttgtgggatttgctggaagggaaagaaaagcctgtgtgtggaacaacctataaagctctaaaggaaattgttgagcgtgttttccagtcaaactactttgatagcactcacaatcatcaaaatgggttgtgtgaggaggaagaggcggcttcagcgcccacagtggaggaccaggtagctgaagctgaacctgagccagcggaagaatacacagagcaaagtgaggttgaatcaacagagtatgtcaataggcagttcatggcagaaacacagttcagcagtggtgagaaggagcaagtggatgagtggacagttgaaacagttgaggttgtaaactcactccagcagcaacctcaggctgcgtccccttcagtcccagagccccactctttgactccagtggctcagtcagatccacttgtgagaaggcagcgtgtacaagatcttatggcacaaatgcaagggccctataatttcatacaggattcaatgttggattttgaaaatcagacgcttgatcctgccattgtatccgcacagcctatgaaccctacccagaacatggatatgcctcagctggtttgccctcaggttcattctgaatctagacttgcccaatctaatcaagttcctgtacaaccagaagccacacaggttcctttggtttcatccacaagtgaggggtatacagcatctcagcccttgtaccagccatctcatgctacggagcagcggccgcagaaagagccaatggatcagattcaggcaacaatatctttgaatacagaccagactacagcatcctcatcccttcctgctgcttctcagcctcaagtgttccaggctgggacaagtaaacctttgcacagcagtggaatcaatgtaaatgcagctccattccagtccatgcaaacggtgttcaatatgaatgctccagtccctcctgctaatgaaccagaaacgttaaaacaacagagtcagtaccaggccacttataaccagagtttttccagtcagcctcaccaagtggaacaaacagagcttcaacaagaccaactgcaaacggtggttggcacttaccatggatcccaggaccagcctcatcaagtgcctggtaaccaccagcaacccccacagcagaacactggctttccacgtagcagtcagccttattacaacagtcgtggggtatctcgaggagggtctcgtggtgccagaggcttgatgaatggatacaggggccctgccaatggatttagaggaggatatgatggttaccgcccttcattctcgaacactccaaacagtggttattcacagtctcagttcactgctccccgggactactctggttaccagcgggatggatatcagcagaatttcaagcgaggctctgggcagagtggaccacggggagccccacgaggtcgtggagggcccccaagacccaacagagggatgccgcaaatgaacactcagcaagtgaattaatgtgatacacaggattatgtttaatcgccaaaaacacactggccagtgtaccataatatgttaccagaagagttattatctatttgttctccctttcaggaaacttattgtaaagggactgttttcatcccataaagacaggactgcaattgtcagctttacattacctggatatggaaggaaactatttttattctgcatgttctgtcctaagcgtcatcttgagccttgcacacaatacaatactcagattcctcacccttgcttaggagtaaaacattatatacttatggggtgataatatctccatagttagttgaagtggcttggaaaaaaaatgcaagattgaatttttgaccttggataaaatctacaatcagccctagaactattcagtggtaattgacaaagttaaagcattttctttgaaaggaagatggaaggagtggagtgtggtttagcaaaactgcatttcatagctttcccattaaattggagcaccgacagattaaaagcataccaaattatgcatgggtccttactcacacaagtgaggctggctaccagccttgacatagcactcactagtcttctggccaaacgactgtgattaaaacacatgtaaattgctctttagtagtggatactgtgtaagacaaagccaaattgcaaatcaggctttgattggctcttctggaaaatatgcatcaaatatgggggataatctggatgggctgctgctgtgctcaatgtgaactatttagatacctttggaacacttaacagtttctctgaacaatgacttacatggggattggtcctgtttgtcattcctcaccataattgcattgtcatcactaatccttggatcttgctgtattgttactcaaattggtaataggtactgatggaaatcgctaatggatggataatcataacacttttggtcacatgttttctcctgcagcctgaaagttcttaaagaaaaagatatcaaatgcctgctgctaccacccttttaaattgctatctttagaaaagcaccggtatgtgttttagattcatttccctgttttagggaaatgacaggcagtagtttcagttctgatggcaaaacaaataaaaacatgtttctaaaagttgtatcttgaaacactggtgttcaacagctagcagctaaagtaattcaacccatgcattgctagtgtcacagcctttggttatgtctagtagctgtttctgaagtattttcatttatcttttgtcaaatttaaccctgtttgaattctctcctttcctcaaggagacacttatgttcaaagtgttgattctttgccttaggtgcatagagagtagacagtttggagatggaaaggttagcagtgacttagccatatgttctgtgttggaatttgtgctagcagtttgagcactagctctgcgtgcctatgaactgaatgctgcttgtcccattccattttatgtcatggagaaataattccacttggtaacacaaaggctaagttaatgttattttctgtacagaaattaaattttacttttagccttttgtaaactttttttttttttttccaagccggtatcagctactcaaaacaattctcagatattcatcattagacaactggagtttttgctggttttgtagcctactaaaactgctgaggctgttgaacattccacattcaaaagttttgtagggtggtggataatggggaagcttcaatgtttattttaaaataaataaaataagttcttgacttttctcatgtgtggttatggtacatcatattggaagggttatctgtttacttttgccaagactattttgccagcacctacacttgtgtgctttaaaagacaactacctgggatgtaccacaaccatatgttaattgtattttattgggatggataaaatgtttgtggtttattggataatccctagatggtgtgttacgtgtgtagaatataattttatgatagtaagaaagcaaaattgaagaaaataagtttagtattgaatttgagttctgaagtgaattcagggaatgtctcacgtttcgggcttctacccaaagtgtagggcagaaggtgtaaaagttgtttgtagtttgacttgtttattttttaagttgcttattcctttcaacagcaacatatcattagctgtcattctaccattgcagttctagtgagttttaacgtctgcattcaagactgttttaaaagcaacctcactggacagagaactgctaaagtcttttccttaagatctgagtctttgttactcagtatcttctataatatgcaaatgcttgtctagaggcagaagaccttttgtttggtcaagtgtgtattttaccagagtacagggaactgatggtcctacatgtctcttagtgtagtaagactataaaatcttttgtacatgcacaattcacagtatgtttagataccacgtgtataatgcccccccctcccccaggtagcatgccattgatgactttttgcttagggccattttattaccagggccttaatattcctaaaaagatgattttttttcatcctttctcctcttttgatcattgtatcttgatattaaaaacatgaccttccaatgattgtagtaaattaacttctatagttcttttgtctctatatgtattcatatatatgctattgtatagagacttcaaggagacatggagatgcatgcttattctcaggttcattcactaaggtgcttggcagacaaccagtttctaagtgcagaatgtagttaagcagcttcatatatgtgccaggcaatttgttttgttaaattttcatctacttaaggaaatagggtattgtagcttaggctgatcatacccttcatttcaaccttaagctctcaacctgcatccatccgacttgagctattaagtactttagttttatcgagtataagttaacagaaaaagtaaattaagctttgcctttactattttgaatttatatacattctggaaaaacttagaaactgttgtatatttcattagattaaattatatgaaaatgtgattgtttatagcaaagcctgtgagttgcatacaccctaaggaaaactccttaagtgctccttgaagagagaagaaacaattctgggtctggtctttttaagaacaaagctagactactgtatgttagcactgtacattaatagtctgttgtgaagcttgagcagtttcctgcatagccttgatccttcaccgttggcattgaaaatagcagtatccctgatgtacttaaaacttaaagtcaggttttggtatatttatttgtaagtcttaatttcctctaaatactatatctctttagcgagacaacctgaaatttattagcacatttgggtatctcttgcttggcattatggccagtgttaactattcagtggtgaaaaaattacccctcaagacactggagtgaccccagatgtgtgtagtaagtggcatggttcaactgtgtggttaatgataaatatatgacttagtcggtatgatctggaaagacttgattgaaagataattcagctgacataaggatgagtgaggagtggcaaactggataaaagagtcaagagacctgtattccagtgactcctgttttgtttaagcattagcaagatctgtctggggaaactggatagggcagttttcttccatgtttagtttttgtctcaacatttggaagctattgaaggttttaaaatggtgtgtattgtttttttttggggggggggtggccagaatagtgggtcatctaataaaactgccatttaaaagatcaaaaaaaaaaaaaaaaaaaaaaaaa

SEQ ID NO: 20 - protein, 707 aa, Mus musculus
MPSATSHSGSGSKSSGPPPPSGSSGSEAAAGAAAPASQHPATGTGAVQTEAMKQILGVIDKKLRNLEKKKGKLDDYQERMNKGERLNQDQLDAVSKYQEVTNNLEFAKELQRSFMALSQDIQKTIKKTARREQLMREEAEQKRLKTVLELQYVLDKLGDDDVRTDLKQGLSGVPILSEEELSLLDEFYKLVDPERDMSLRLNEQYEHASIHLWDLLEGKEKPVCGTTYKALKEIVERVFQSNYFDSTHNHQNGLCEEEEAASAPTVEDQVAEAEPEPAEEYTEQSEVESTEYVNRQFMAETQFSSGEKEQVDEWTVETVEVVNSLQQQPQAASPSVPEPHSLTPVAQSDPLVRRQRVQDLMAQMQGPYNFIQDSMLDFENQTLDPAIVSAQPMNPTQNMDMPQLVCPQVHSESRLAQSNQVPVQPEATQVPLVSSTSEGYTASQPLYQPSHATEQRPQKEPMDQIQATISLNTDQTTASSSLPAASQPQVFQAGTSKPLHSSGINVNAAPFQSMQTVFNMNAPVPPANEPETLKQQSQYQATYNQSFSSQPHQVEQTELQQDQLQTVVGTYHGSQDQPHQVPGNHQQPPQQNTGFPRSSQPYYNSRGVSRGGSRGARGLMNGYRGPANGFRGGYDGYRPSFSNTPNSGYSQSQFTAPRDYSGYQRDGYQQNFKRGSGQSGPRGAPRGRGGPPRPNRGMPQMNTQQVN

SEQ ID NO: 21 - DNA, 6141 bp, Mus musculus
  source 1..6141: mol_type = other DNA
  CDS 139..2262: protein_id = 320; translation = MPSATSHSGSGSKSSGPPPPSGSSGSEAAAGAAAPASQHPATGTGAVQTEAMKQILGVIDKKLRNLEKKKGKLDDYQERMNKGERLNQDQLDAVSKYQEVTNNLEFAKELQRSFMALSQDIQKTIKKTARREQLMREEAEQKRLKTVLELQYVLDKLGDDDVRTDLKQGLSGVPILSEEELSLLDEFYKLVDPERDMSLRLNEQYEHASIHLWDLLEGKEKPVCGTTYKALKEIVERVFQSNYFDSTHNHQNGLCEEEEAASAPTVEDQVAEAEPEPAEEYTEQSEVESTEYVNRQFMAETQFSSGEKEQVDEWTVETVEVVNSLQQQPQAASPSVPEPHSLTPVAQSDPLVRRQRVQDLMAQMQGPYNFIQDSMLDFENQTLDPAIVSAQPMNPTQNMDMPQLVCPQVHSESRLAQSNQVPVQPEATQVPLVSSTSEGYTASQPLYQPSHATEQRPQKEPMDQIQATISLNTDQTTASSSLPAASQPQVFQAGTSKPLHSSGINVNAAPFQSMQTVFNMNAPVPPANEPETLKQQSQYQATYNQSFSSQPHQVEQTELQQDQLQTVVGTYHGSQDQPHQVPGNHQQPPQQNTGFPRSSQPYYNSRGVSRGGSRGARGLMNGYRGPANGFRGGYDGYRPSFSNTPNSGYSQSQFTAPRDYSGYQRDGYQQNFKRGSGQSGPRGAPRGRGGPPRPNRGMPQMNTQQVN
cccaccgcgcgcgcgcgtagccgcctgcccgcccgcccgctgcgcgttttgtcccgcgtctctccccgtccgtctcctgacttgctggtcttgtccttccctcccgcttttttcctctcctctcttctcggtctaaagatgccctcggccaccagccacagcggaagcggcagcaaatcgtcgggaccgccgccgccgtccggttcctccgggagtgaggcggcggccggggcagctgcgccggcttctcagcatccggcaaccggcaccggcgccgtccagaccgaggccatgaagcagattctcggcgtaatcgacaagaaacttcggaacctggagaagaaaaagggtaaacttgatgattaccaggaacgaatgaataaaggggaaaggctcaatcaagaccagctggatgccgtatctaagtaccaggaagtcacaaataatttggagtttgcaaaggaattacagaggagtttcatggcattaagtcaagatattcagaaaacaataaagaagacagcacgtcgggaacagcttatgagagaagaagcagaacagaagcgcttaaaaactgtacttgagttacagtatgtattggataagctgggagatgatgatgtgagaacagatctgaaacaaggtttgagtggagtgccaatattgtctgaggaggagttgtcattgctggatgagttctacaagctcgtagatcctgagcgtgacatgagtttaaggttaaatgagcagtatgaacatgcctcaattcacttgtgggatttgctggaagggaaagaaaagcctgtgtgtggaacaacctataaagctctaaaggaaattgttgagcgtgttttccagtcaaactactttgatagcactcacaatcatcaaaatgggttgtgtgaggaggaagaggcggcttcagcgcccacagtggaggaccaggtagctgaagctgaacctgagccagcggaagaatacacagagcaaagtgaggttgaatcaacagagtatgtcaataggcagttcatggcagaaacacagttcagcagtggtgagaaggagcaagtggatgagtggacagttgaaacagttgaggttgtaaactcactccagcagcaacctcaggctgcgtccccttcagtcccagagccccactctttgactccagtggctcagtcagatccacttgtgagaaggcagcgtgtacaagatcttatggcacaaatgcaagggccctataatttcatacaggattcaatgttggattttgaaaatcagacgcttgatcctgccattgtatccgcacagcctatgaaccctacccagaacatggatatgcctcagctggtttgccctcaggttcattctgaatctagacttgcccaatctaatcaagttcctgtacaaccagaagccacacaggttcctttggtttcatccacaagtgaggggtatacagcatctcagcccttgtaccagccatctcatgctacggagcagcggccgcagaaagagccaatggatcagattcaggcaacaatatctttgaatacagaccagactacagcatcctcatcccttcctgctgcttctcagcctcaagtgttccaggctgggacaagtaaacctttgcacagcagtggaatcaatgtaaatgcagctccattccagtccatgcaaacggtgttcaatatgaatgctccagtccctcctgctaatgaaccagaaacgttaaaacaacagagtcagtaccaggccacttataaccagagtttttccagtcagcctcaccaagtggaacaaacagagcttcaacaagaccaactgcaaacggtggttggcacttaccatggatcccaggaccagcctcatcaagtgcctggtaaccaccagcaacccccacagcagaacactggctttccacgtagcagtcagccttattacaacagtcgtggggtatctcgaggagggtctcgtggtgccagaggcttgatgaatggatacaggggccctgccaatggatttagaggaggatatgatggttaccgcccttcattctcgaacactccaaacagtggttattcacagtctcagttcactgctccccgggactactctggttaccagcgggatggatatcagcagaatttcaagcgaggctctgggcagagtggaccacggggagccccacgaggtcgtggagggcccccaagacccaacagagggatgccgcaaatgaacactcagcaagtgaattaatgtgatacacaggattatgtttaatcgccaaaaacacactggccagtgtaccataatatgttaccagaagagttattatctatttgttctccctttcaggaaacttattgtaaagggactgttttcatcccataaagacaggactgcaattgtcagctttacattacctggatatggaaggaaactatttttattctgcatgttctgtcctaagcgtcatcttgagccttgcacacaatacaatactcagattcctcacccttgcttaggagtaaaacattatatacttatggggtgataatatctccatagttagttgaagtggcttggaaaaaaaatgcaagattgaatttttgaccttggataaaatctacaatcagccctagaactattcagtggtaattgacaaagttaaagcattttctttgaaaggaagatggaaggagtggagtgtggtttagcaaaactgcatttcatagctttcccattaaattggagcaccgacagattaaaagcataccaaattatgcatgggtccttactcacacaagtgaggctggctaccagccttgacatagcactcactagtcttctggccaaacgactgtgattaaaacacatgtaaattgctctttagtagtggatactgtgtaagacaaagccaaattgcaaatcaggctttgattggctcttctggaaaatatgcatcaaatatgggggataatctggatgggctgctgctgtgctcaatgtgaactatttagatacctttggaacacttaacagtttctctgaacaatgacttacatggggattggtcctgtttgtcattcctcaccataattgcattgtcatcactaatccttggatcttgctgtattgttactcaaattggtaataggtactgatggaaatcgctaatggatggataatcataacacttttggtcacatgttttctcctgcagcctgaaagttcttaaagaaaaagatatcaaatgcctgctgctaccacccttttaaattgctatctttagaaaagcaccggtatgtgttttagattcatttccctgttttagggaaatgacaggcagtagtttcagttctgatggcaaaacaaataaaaacatgtttctaaaagttgtatcttgaaacactggtgttcaacagctagcagctaaagtaattcaacccatgcattgctagtgtcacagcctttggttatgtctagtagctgtttctgaagtattttcatttatcttttgtcaaatttaaccctgtttgaattctctcctttcctcaaggagacacttatgttcaaagtgttgattctttgccttaggtgcatagagagtagacagtttggagatggaaaggttagcagtgacttagccatatgttctgtgttggaatttgtgctagcagtttgagcactagctctgcgtgcctatgaactgaatgctgcttgtcccattccattttatgtcatggagaaataattccacttggtaacacaaaggctaagttaatgttattttctgtacagaaattaaattttacttttagccttttgtaaactttttttttttttttccaagccggtatcagctactcaaaacaattctcagatattcatcattagacaactggagtttttgctggttttgtagcctactaaaactgctgaggctgttgaacattccacattcaaaagttttgtagggtggtggataatggggaagcttcaatgtttattttaaaataaataaaataagttcttgacttttctcatgtgtggttatggtacatcatattggaagggttatctgtttacttttgccaagactattttgccagcacctacacttgtgtgctttaaaagacaactacctgggatgtaccacaaccatatgttaattgtattttattgggatggataaaatgtttgtggtttattggataatccctagatggtgtgttacgtgtgtagaatataattttatgatagtaagaaagcaaaattgaagaaaataagtttagtattgaatttgagttctgaagtgaattcagggaatgtctcacgtttcgggcttctacccaaagtgtagggcagaaggtgtaaaagttgtttgtagtttgacttgtttattttttaagttgcttattcctttcaacagcaacatatcattagctgtcattctaccattgcagttctagtgagttttaacgtctgcattcaagactgttttaaaagcaacctcactggacagagaactgctaaagtcttttccttaagatctgagtctttgttactcagtatcttctataatatgcaaatgcttgtctagaggcagaagaccttttgtttggtcaagtgtgtattttaccagagtacagggaactgatggtcctacatgtctcttagtgtagtaagactataaaatcttttgtacatgcacaattcacagtatgtttagataccacgtgtataatgcccccccctcccccaggtagcatgccattgatgactttttgcttagggccattttattaccagggccttaatattcctaaaaagatgattttttttcatcctttctcctcttttgatcattgtatcttgatattaaaaacatgaccttccaatgattgtagtaaattaacttctatagttcttttgtctctatatgtattcatatatatgctattgtatagagacttcaaggagacatggagatgcatgcttattctcaggttcattcactaaggtgcttggcagacaaccagtttctaagtgcagaatgtagttaagcagcttcatatatgtgccaggcaatttgttttgttaaattttcatctacttaaggaaatagggtattgtagcttaggctgatcatacccttcatttcaaccttaagctctcaacctgcatccatccgacttgagctattaagtactttagttttatcgagtataagttaacagaaaaagtaaattaagctttgcctttactattttgaatttatatacattctggaaaaacttagaaactgttgtatatttcattagattaaattatatgaaaatgtgattgtttatagcaaagcctgtgagttgcatacaccctaaggaaaactccttaagtgctccttgaagagagaagaaacaattctgggtctggtctttttaagaacaaagctagactactgtatgttagcactgtacattaatagtctgttgtgaagcttgagcagtttcctgcatagccttgatccttcaccgttggcattgaaaatagcagtatccctgatgtacttaaaacttaaagtcaggttttggtatatttatttgtaagtcttaatttcctctaaatactatatctctttagcgagacaacctgaaatttattagcacatttgggtatctcttgcttggcattatggccagtgttaactattcagtggtgaaaaaattacccctcaagacactggagtgaccccagatgtgtgtagtaagtggcatggttcaactgtgtggttaatgataaatatatgacttagtcggtatgatctggaaagacttgattgaaagataattcagctgacataaggatgagtgaggagtggcaaactggataaaagagtcaagagacctgtattccagtgactcctgttttgtttaagcattagcaagatctgtctggggaaactggatagggcagttttcttccatgtttagtttttgtctcaacatttggaagctattgaaggttttaaaatggtgtgtattgtttttttttggggggggggtggccagaatagtgggtcatctaataaaactgccatttaaaagatcaaaaaaaaaaaaaaaaaaaaaaaaa

SEQ ID NO: 22 - protein, 707 aa, Mus musculus; identical to SEQ ID NO: 20

SEQ ID NO: 23 - DNA, 6114 bp, Mus musculus
  source 1..6114: mol_type = other DNA
  CDS 139..2235: protein_id = 321; translation = MPSATSHSGSGSKSSGPPPPSGSSGSEAAAGAAAPASQHPATGTGAVQTEAMKQILGVIDKKLRNLEKKKGKLDDYQERMNKGERLNQDQLDAVSKYQEVTNNLEFAKELQRSFMALSQDIQKTIKKTARREQLMREEAEQKRLKTVLELQYVLDKLGDDDVRTDLKQGLSGVPILSEEELSLLDEFYKLVDPERDMSLRLNEQYEHASIHLWDLLEGKEKPVCGTTYKALKEIVERVFQSNYFDSTHNHQNGLCEEEEAASAPTVEDQVAEAEPEPAEEYTEQSEVESTEYVNRQFMAETQFSSGEKEQVDEWTVETVEVVNSLQQQPQAASPSVPEPHSLTPVAQSDPLVRRQRVQDLMAQMQGPYNFIQTLDPAIVSAQPMNPTQNMDMPQLVCPQVHSESRLAQSNQVPVQPEATQVPLVSSTSEGYTASQPLYQPSHATEQRPQKEPMDQIQATISLNTDQTTASSSLPAASQPQVFQAGTSKPLHSSGINVNAAPFQSMQTVFNMNAPVPPANEPETLKQQSQYQATYNQSFSSQPHQVEQTELQQDQLQTVVGTYHGSQDQPHQVPGNHQQPPQQNTGFPRSSQPYYNSRGVSRGGSRGARGLMNGYRGPANGFRGGYDGYRPSFSNTPNSGYSQSQFTAPRDYSGYQRDGYQQNFKRGSGQSGPRGAPRGRGGPPRPNRGMPQMNTQQVN
cccaccgcgcgcgcgcgtagccgcctgcccgcccgcccgctgcgcgttttgtcccgcgtctctccccgtccgtctcctgacttgctggtcttgtccttccctcccgcttttttcctctcctctcttctcggtctaaagatgccctcggccaccagccacagcggaagcggcagcaaatcgtcgggaccgccgccgccgtccggttcctccgggagtgaggcggcggccggggcagctgcgccggcttctcagcatccggcaaccggcaccggcgccgtccagaccgaggccatgaagcagattctcggcgtaatcgacaagaaacttcggaacctggagaagaaaaagggtaaacttgatgattaccaggaacgaatgaataaaggggaaaggctcaatcaagaccagctggatgccgtatctaagtaccaggaagtcacaaataatttggagtttgcaaaggaattacagaggagtttcatggcattaagtcaagatattcagaaaacaataaagaagacagcacgtcgggaacagcttatgagagaagaagcagaacagaagcgcttaaaaactgtacttgagttacagtatgtattggataagctgggagatgatgatgtgagaacagatctgaaacaaggtttgagtggagtgccaatattgtctgaggaggagttgtcattgctggatgagttctacaagctcgtagatcctgagcgtgacatgagtttaaggttaaatgagcagtatgaacatgcctcaattcacttgtgggatttgctggaagggaaagaaaagcctgtgtgtggaacaacctataaagctctaaaggaaattgttgagcgtgttttccagtcaaactactttgatagcactcacaatcatcaaaatgggttgtgtgaggaggaagaggcggcttcagcgcccacagtggaggaccaggtagctgaagctgaacctgagccagcggaagaatacacagagcaaagtgaggttgaatcaacagagtatgtcaataggcagttcatggcagaaacacagttcagcagtggtgagaaggagcaagtggatgagtggacagttgaaacagttgaggttgtaaactcactccagcagcaacctcaggctgcgtccccttcagtcccagagccccactctttgactccagtggctcagtcagatccacttgtgagaaggcagcgtgtacaagatcttatggcacaaatgcaagggccctataatttcatacagacgcttgatcctgccattgtatccgcacagcctatgaaccctacccagaacatggatatgcctcagctggtttgccctcaggttcattctgaatctagacttgcccaatctaatcaagttcctgtacaaccagaagccacacaggttcctttggtttcatccacaagtgaggggtatacagcatctcagcccttgtaccagccatctcatgctacggagcagcggccgcagaaagagccaatggatcagattcaggcaacaatatctttgaatacagaccagactacagcatcctcatcccttcctgctgcttctcagcctcaagtgttccaggctgggacaagtaaacctttgcacagcagtggaatcaatgtaaatgcagctccattccagtccatgcaaacggtgttcaatatgaatgctccagtccctcctgctaatgaaccagaaacgttaaaacaacagagtcagtaccaggccacttataaccagagtttttccagtcagcctcaccaagtggaacaaacagagcttcaacaagaccaactgcaaacggtggttggcacttaccatggatcccaggaccagcctcatcaagtgcctggtaaccaccagcaacccccacagcagaacactggctttccacgtagcagtcagccttattacaacagtcgtggggtatctcgaggagggtctcgtggtgccagaggcttgatgaatggatacaggggccctgccaatggatttagaggaggatatgatggttaccgcccttcattctcgaacactccaaacagtggttattcacagtctcagttcactgctccccgggactactctggttaccagcgggatggatatcagcagaatttcaagcgaggctctgggcagagtggaccacggggagccccacgaggtcgtggagggcccccaagacccaacagagggatgccgcaaatgaacactcagcaagtgaattaatgtgatacacaggattatgtttaatcgccaaaaacacactggccagtgtaccataatatgttaccagaagagttattatctatttgttctccctttcaggaaacttattgtaaagggactgttttcatcccataaagacaggactgcaattgtcagctttacattacctggatatggaaggaaactatttttattctgcatgttctgtcctaagcgtcatcttgagccttgcacacaatacaatactcagattcctcacccttgcttaggagtaaaacattatatacttatggggtgataatatctccatagttagttgaagtggcttggaaaaaaaatgcaagattgaatttttgaccttggataaaatctacaatcagccctagaactattcagtggtaattgacaaagttaaagcattttctttgaaaggaagatggaaggagtggagtgtggtttagcaaaactgcatttcatagctttcccattaaattggagcaccgacagattaaaagcataccaaattatgcatgggtccttactcacacaagtgaggctggctaccagccttgacatagcactcactagtcttctggccaaacgactgtgattaaaacacatgtaaattgctctttagtagtggatactgtgtaagacaaagccaaattgcaaatcaggctttgattggctcttctggaaaatatgcatcaaatatgggggataatctggatgggctgctgctgtgctcaatgtgaactatttagatacctttggaacacttaacagtttctctgaacaatgacttacatggggattggtcctgtttgtcattcctcaccataattgcattgtcatcactaatccttggatcttgctgtattgttactcaaattggtaataggtactgatggaaatcgctaatggatggataatcataacacttttggtcacatgttttctcctgcagcctgaaagttcttaaagaaaaagatatcaaatgcctgctgctaccacccttttaaattgctatctttagaaaagcaccggtatgtgttttagattcatttccctgttttagggaaatgacaggcagtagtttcagttctgatggcaaaacaaataaaaacatgtttctaaaagttgtatcttgaaacactggtgttcaacagctagcagctaaagtaattcaacccatgcattgctagtgtcacagcctttggttatgtctagtagctgtttctgaagtattttcatttatcttttgtcaaatttaaccctgtttgaattctctcctttcctcaaggagacacttatgttcaaagtgttgattctttgccttaggtgcatagagagtagacagtttggagatggaaaggttagcagtgacttagccatatgttctgtgttggaatttgtgctagcagtttgagcactagctctgcgtgcctatgaactgaatgctgcttgtcccattccattttatgtcatggagaaataattccacttggtaacacaaaggctaagttaatgttattttctgtacagaaattaaattttacttttagccttttgtaaactttttttttttttttccaagccggtatcagctactcaaaacaattctcagatattcatcattagacaactggagtttttgctggttttgtagcctactaaaactgctgaggctgttgaacattccacattcaaaagttttgtagggtggtggataatggggaagcttcaatgtttattttaaaataaataaaataagttcttgacttttctcatgtgtggttatggtacatcatattggaagggttatctgtttacttttgccaagactattttgccagcacctacacttgtgtgctttaaaagacaactacctgggatgtaccacaaccatatgttaattgtattttattgggatggataaaatgtttgtggtttattggataatccctagatggtgtgttacgtgtgtagaatataattttatgatagtaagaaagcaaaattgaagaaaataagtttagtattgaatttgagttctgaagtgaattcagggaatgtctcacgtttcgggcttctacccaaagtgtagggcagaaggtgtaaaagttgtttgtagtttgacttgtttattttttaagttgcttattcctttcaacagcaacatatcattagctgtcattctaccattgcagttctagtgagttttaacgtctgcattcaagactgttttaaaagcaacctcactggacagagaactgctaaagtcttttccttaagatctgagtctttgttactcagtatcttctataatatgcaaatgcttgtctagaggcagaagaccttttgtttggtcaagtgtgtattttaccagagtacagggaactgatggtcctacatgtctcttagtgtagtaagactataaaatcttttgtacatgcacaattcacagtatgtttagataccacgtgtataatgcccccccctcccccaggtagcatgccattgatgactttttgcttagggccattttattaccagggccttaatattcctaaaaagatgattttttttcatcctttctcctcttttgatcattgtatcttgatattaaaaacatgaccttccaatgattgtagtaaattaacttctatagttcttttgtctctatatgtattcatatatatgctattgtatagagacttcaaggagacatggagatgcatgcttattctcaggttcattcactaaggtgcttggcagacaaccagtttctaagtgcagaatgtagttaagcagcttcatatatgtgccaggcaatttgttttgttaaattttcatctacttaaggaaatagggtattgtagcttaggctgatcatacccttcatttcaaccttaagctctcaacctgcatccatccgacttgagctattaagtactttagttttatcgagtataagttaacagaaaaagtaaattaagctttgcctttactattttgaatttatatacattctggaaaaacttagaaactgttgtatatttcattagattaaattatatgaaaatgtgattgtttatagcaaagcctgtgagttgcatacaccctaaggaaaactccttaagtgctccttgaagagagaagaaacaattctgggtctggtctttttaagaacaaagctagactactgtatgttagcactgtacattaatagtctgttgtgaagcttgagcagtttcctgcatagccttgatccttcaccgttggcattgaaaatagcagtatccctgatgtacttaaaacttaaagtcaggttttggtatatttatttgtaagtcttaatttcctctaaatactatatctctttagcgagacaacctgaaatttattagcacatttgggtatctcttgcttggcattatggccagtgttaactattcagtggtgaaaaaattacccctcaagacactggagtgaccccagatgtgtgtagtaagtggcatggttcaactgtgtggttaatgataaatatatgacttagtcggtatgatctggaaagacttgattgaaagataattcagctgacataaggatgagtgaggagtggcaaactggataaaagagtcaagagacctgtattccagtgactcctgttttgtttaagcattagcaagatctgtctggggaaactggatagggcagttttcttccatgtttagtttttgtctcaacatttggaagctattgaaggttttaaaatggtgtgtattgtttttttttggggggggggtggccagaatagtgggtcatctaataaaactgccatttaaaagatcaaaaaaaaaaaaaaaaaaaaaaaaa

SEQ ID NO: 24 - protein, 698 aa, Mus musculus
MPSATSHSGSGSKSSGPPPPSGSSGSEAAAGAAAPASQHPATGTGAVQTEAMKQILGVIDKKLRNLEKKKGKLDDYQERMNKGERLNQDQLDAVSKYQEVTNNLEFAKELQRSFMALSQDIQKTIKKTARREQLMREEAEQKRLKTVLELQYVLDKLGDDDVRTDLKQGLSGVPILSEEELSLLDEFYKLVDPERDMSLRLNEQYEHASIHLWDLLEGKEKPVCGTTYKALKEIVERVFQSNYFDSTHNHQNGLCEEEEAASAPTVEDQVAEAEPEPAEEYTEQSEVESTEYVNRQFMAETQFSSGEKEQVDEWTVETVEVVNSLQQQPQAASPSVPEPHSLTPVAQSDPLVRRQRVQDLMAQMQGPYNFIQTLDPAIVSAQPMNPTQNMDMPQLVCPQVHSESRLAQSNQVPVQPEATQVPLVSSTSEGYTASQPLYQPSHATEQRPQKEPMDQIQATISLNTDQTTASSSLPAASQPQVFQAGTSKPLHSSGINVNAAPFQSMQTVFNMNAPVPPANEPETLKQQSQYQATYNQSFSSQPHQVEQTELQQDQLQTVVGTYHGSQDQPHQVPGNHQQPPQQNTGFPRSSQPYYNSRGVSRGGSRGARGLMNGYRGPANGFRGGYDGYRPSFSNTPNSGYSQSQFTAPRDYSGYQRDGYQQNFKRGSGQSGPRGAPRGRGGPPRPNRGMPQMNTQQVN

SEQ ID NO: 25 - DNA, 3548 bp, Mus musculus
  source 1..3548: mol_type = other DNA
  CDS 179..2257: protein_id = 322; translation = MPSATSHSGSGSKSSGPPPPSGSSGSEAAAGAAAPASQHPATGTGAVQTEAMKQILGVIDKKLRNLEKKKGKLDDYQERMNKGERLNQDQLDAVSKYQEVTNNLEFAKELQRSFMALSQDIQKTIKKTARREQLMREEAEQKRLKTVLELQYVLDKLGDDDVRTDLKQGLSGVPILSEEELSLLDEFYKLVDPERDMSLRLNEQYEHASIHLWDLLEGKEKPVCGTTYKALKEIVERVFQSNYFDSTHNHQNGLCEEEEAASAPTVEDQVAEAEPEPAEEYTEQSEVESTEYVNRQFMAETQFSSGEKEQVDEWTVETVEVVNSLQQQPQAASPSVPEPHSLTPVAQSDPLVRRQRVQDLMAQMQGPYNFIQDSMLDFENQTLDPAIVSAQPMNPTQNMDMPQLVCPQVHSESRLAQSNQVPVQPEATQVPLVSSTSEGYTASQPLYQPSHATEQRPQKEPMDQIQATISLNTDQTTASSSLPAASQPQVFQAGTSKPLHSSGINVNAAPFQSMQTVFNMNAPVPPANEPETLKQQSQYQATYNQSFSSQPHQVEQTELQQDQLQTVVGTYHGSQDQPHQVPGNHQQPPQQNTGFPRSSQPYYNSRGVSRGGSRGARGLMNGYRGPANGFRGGYDGYRPSFSNTPNSGYSQSQFTAPRDYSGYQRDGYQQNFKRGSGQSGPRGAPRGNILWW
gctggctggctaagtccctcccgcgccggctcttgtcccactaggagcagctcagagccgcggggacagggcgaagcggcctgcgcccacggagcgcacgtctctgttctcaacgcagcaccacccttgcccccctcggctgcccactccagacgtccagcggctccgcgcgcgcacgatgccctcggccaccagccacagcggaagcggcagcaaatcgtcgggaccgccgccgccgtccggttcctccgggagtgaggcggcggccggggcagctgcgccggcttctcagcatccggcaaccggcaccggcgccgtccagaccgaggccatgaagcagattctcggcgtaatcgacaagaaacttcggaacctggagaagaaaaagggtaaacttgatgattaccaggaacgaatgaataaaggggaaaggctcaatcaagaccagctggatgccgtatctaagtaccaggaagtcacaaataatttggagtttgcaaaggaattacagaggagtttcatggcattaagtcaagatattcagaaaacaataaagaagacagcacgtcgggaacagcttatgagagaagaagcagaacagaagcgcttaaaaactgtacttgagttacagtatgtattggataagctgggagatgatgatgtgagaacagatctgaaacaaggtttgagtggagtgccaatattgtctgaggaggagttgtcattgctggatgagttctacaagctcgtagatcctgagcgtgacatgagtttaaggttaaatgagcagtatgaacatgcctcaattcacttgtgggatttgctggaagggaaagaaaagcctgtgtgtggaacaacctataaagctctaaaggaaattgttgagcgtgttttccagtcaaactactttgatagcactcacaatcatcaaaatgggttgtgtgaggaggaagaggcggcttcagcgcccacagtggaggaccaggtagctgaagctgaacctgagccagcggaagaatacacagagcaaagtgaggttgaatcaacagagtatgtcaataggcagttcatggcagaaacacagttcagcagtggtgagaaggagcaagtggatgagtggacagttgaaacagttgaggttgtaaactcactccagcagcaacctcaggctgcgtccccttcagtcccagagccccactctttgactccagtggctcagtcagatccacttgtgagaaggcagcgtgtacaagatcttatggcacaaatgcaagggccctataatttcatacaggattcaatgttggattttgaaaatcagacgcttgatcctgccattgtatccgcacagcctatgaaccctacccagaacatggatatgcctcagctggtttgccctcaggttcattctgaatctagacttgcccaatctaatcaagttcctgtacaaccagaagccacacaggttcctttggtttcatccacaagtgaggggtatacagcatctcagcccttgtaccagccatctcatgctacggagcagcggccgcagaaagagccaatggatcagattcaggcaacaatatctttgaatacagaccagactacagcatcctcatcccttcctgctgcttctcagcctcaagtgttccaggctgggacaagtaaacctttgcacagcagtggaatcaatgtaaatgcagctccattccagtccatgcaaacggtgttcaatatgaatgctccagtccctcctgctaatgaaccagaaacgttaaaacaacagagtcagtaccaggccacttataaccagagtttttccagtcagcctcaccaagtggaacaaacagagcttcaacaagaccaactgcaaacggtggttggcacttaccatggatcccaggaccagcctcatcaagtgcctggtaaccaccagcaacccccacagcagaacactggctttccacgtagcagtcagccttattacaacagtcgtggggtatctcgaggagggtctcgtggtgccagaggcttgatgaatggatacaggggccctgccaatggatttagaggaggatatgatggttaccgcccttcattctcgaacactccaaacagtggttattcacagtctcagttcactgctccccgggactactctggttaccagcgggatggatatcagcagaatttcaagcgaggctctgggcagagtggaccacggggagccccacgaggtaatatattgtggtggtgatcctagctcctatgtggagcttctgttctggccttggaagaactgttcatagtccgcatgtaggttacatgttaggaatacatttatcttttccagacttgttgctaaagattaaatgaaatgctctgtttctaaaatttcatcttgaatccaaattttaatttttgaatgactttccctgctgttgtcttcaaaatcagaacattttctctgcctcagaaaagcgtttttccaactggaaatttatttttcaggtcttaaaacctgctaaatgtttttaggaagtacctactgaaactttttgtaagacatttttggaacgagcttgaacatttatataaatttattaccctctttgatttttgaaacatgcatattatatttaggctgagaagcccttcaaatggccagataagccacagttttagctagagaaccatttagaattgacataactaatctaaacttgaacacttttaggaccaatgttagtgttctaaataccaacatatttctgatgtttaaacagatctcccaaattcttaggaccttgatgtcattaaaatttagaatgacaagcttaagaggctttagtttcatttgtttttcaagtaatgaaaaataatttcttacatgggcagatagttaatttgttgaacaattacaggtagcatttcatgtaatctgatgttctaaatggttctcttattgaaggaggttaaagaattaggtttcttacagtttttggctggccatgacatgtataaaatgtatattaaggaggaattataaagtactttaatttgaatgctagtggcaattgatcattaagaaagtactttaaagcaaaaggttaatgggtcatctgggaaaaatactgaagtatcaaaggtatttgcatgtgaatgtgggttatgttcttctatcccaccttgtagcatattctatgaaagttgagttaaatgatagctaaaatatctgtttcaacagcatgtaaaaagttattttaactgttacaagtcattatacaattttgaatgttctgtagtttctttttaacagtttaggtacaaaggtctgttttcattctggtgctttttattaattttgatagtatgatgtcacttcctattgaaatgtaagctagcgtgtaccttagaatgtgagctccatgagagcaggtaccttgtttgtcttcactgctgtatctattcccaacgcctcatgacagtgcctggcacatagtaggcactcaataaatacttgttgaatgaatgaaaaaaaaaaaaaa

SEQ ID NO: 26 - protein, 692 aa, Mus musculus
MPSATSHSGSGSKSSGPPPPSGSSGSEAAAGAAAPASQHPATGTGAVQTEAMKQILGVIDKKLRNLEKKKGKLDDYQERMNKGERLNQDQLDAVSKYQEVTNNLEFAKELQRSFMALSQDIQKTIKKTARREQLMREEAEQKRLKTVLELQYVLDKLGDDDVRTDLKQGLSGVPILSEEELSLLDEFYKLVDPERDMSLRLNEQYEHASIHLWDLLEGKEKPVCGTTYKALKEIVERVFQSNYFDSTHNHQNGLCEEEEAASAPTVEDQVAEAEPEPAEEYTEQSEVESTEYVNRQFMAETQFSSGEKEQVDEWTVETVEVVNSLQQQPQAASPSVPEPHSLTPVAQSDPLVRRQRVQDLMAQMQGPYNFIQDSMLDFENQTLDPAIVSAQPMNPTQNMDMPQLVCPQVHSESRLAQSNQVPVQPEATQVPLVSSTSEGYTASQPLYQPSHATEQRPQKEPMDQIQATISLNTDQTTASSSLPAASQPQVFQAGTSKPLHSSGINVNAAPFQSMQTVFNMNAPVPPANEPETLKQQSQYQATYNQSFSSQPHQVEQTELQQDQLQTVVGTYHGSQDQPHQVPGNHQQPPQQNTGFPRSSQPYYNSRGVSRGGSRGARGLMNGYRGPANGFRGGYDGYRPSFSNTPNSGYSQSQFTAPRDYSGYQRDGYQQNFKRGSGQSGPRGAPRGNILWW

SEQ ID NO: 27 - DNA, 3508 bp, Mus musculus
  source 1..3508: mol_type = other DNA
  CDS 139..2217: protein_id = 323; translation = MPSATSHSGSGSKSSGPPPPSGSSGSEAAAGAAAPASQHPATGTGAVQTEAMKQILGVIDKKLRNLEKKKGKLDDYQERMNKGERLNQDQLDAVSKYQEVTNNLEFAKELQRSFMALSQDIQKTIKKTARREQLMREEAEQKRLKTVLELQYVLDKLGDDDVRTDLKQGLSGVPILSEEELSLLDEFYKLVDPERDMSLRLNEQYEHASIHLWDLLEGKEKPVCGTTYKALKEIVERVFQSNYFDSTHNHQNGLCEEEEAASAPTVEDQVAEAEPEPAEEYTEQSEVESTEYVNRQFMAETQFSSGEKEQVDEWTVETVEVVNSLQQQPQAASPSVPEPHSLTPVAQSDPLVRRQRVQDLMAQMQGPYNFIQDSMLDFENQTLDPAIVSAQPMNPTQNMDMPQLVCPQVHSESRLAQSNQVPVQPEATQVPLVSSTSEGYTASQPLYQPSHATEQRPQKEPMDQIQATISLNTDQTTASSSLPAASQPQVFQAGTSKPLHSSGINVNAAPFQSMQTVFNMNAPVPPANEPETLKQQSQYQATYNQSFSSQPHQVEQTELQQDQLQTVVGTYHGSQDQPHQVPGNHQQPPQQNTGFPRSSQPYYNSRGVSRGGSRGARGLMNGYRGPANGFRGGYDGYRPSFSNTPNSGYSQSQFTAPRDYSGYQRDGYQQNFKRGSGQSGPRGAPRGNILWW
cccaccgcgcgcgcgcgtagccgcctgcccgcccgcccgctgcgcgttttgtcccgcgtctctccccgtccgtctcctgacttgctggtcttgtccttccctcccgcttttttcctctcctctcttctcggtctaaagatgccctcggccaccagccacagcggaagcggcagcaaatcgtcgggaccgccgccgccgtccggttcctccgggagtgaggcggcggccggggcagctgcgccggcttctcagcatccggcaaccggcaccggcgccgtccagaccgaggccatgaagcagattctcggcgtaatcgacaagaaacttcggaacctggagaagaaaaagggtaaacttgatgattaccaggaacgaatgaataaaggggaaaggctcaatcaagaccagctggatgccgtatctaagtaccaggaagtcacaaataatttggagtttgcaaaggaattacagaggagtttcatggcattaagtcaagatattcagaaaacaataaagaagacagcacgtcgggaacagcttatgagagaagaagcagaacagaagcgcttaaaaactgtacttgagttacagtatgtattggataagctgggagatgatgatgtgagaacagatctgaaacaaggtttgagtggagtgccaatattgtctgaggaggagttgtcattgctggatgagttctacaagctcgtagatcctgagcgtgacatgagtttaaggttaaatgagcagtatgaacatgcctcaattcacttgtgggatttgctggaagggaaagaaaagcctgtgtgtggaacaacctataaagctctaaaggaaattgttgagcgtgttttccagtcaaactactttgatagcactcacaatcatcaaaatgggttgtgtgaggaggaagaggcggcttcagcgcccacagtggaggaccaggtagctgaagctgaacctgagccagcggaagaatacacagagcaaagtgaggttgaatcaacagagtatgtcaataggcagttcatggcagaaacacagttcagcagtggtgagaaggagcaagtggatgagtggacagttgaaacagttgaggttgtaaactcactccagcagcaacctcaggctgcgtccccttcagtcccagagccccactctttgactccagtggctcagtcagatccacttgtgagaaggcagcgtgtacaagatcttatggcacaaatgcaagggccctataatttcatacaggattcaatgttggattttgaaaatcagacgcttgatcctgccattgtatccgcacagcctatgaaccctacccagaacatggatatgcctcagctggtttgccctcaggttcattctgaatctagacttgcccaatctaatcaagttcctgtacaaccagaagccacacaggttcctttggtttcatccacaagtgaggggtatacagcatctcagcccttgtaccagccatctcatgctacggagcagcggccgcagaaagagccaatggatcagattcaggcaacaatatctttgaatacagaccagactacagcatcctcatcccttcctgctgcttctcagcctcaagtgttccaggctgggacaagtaaacctttgcacagcagtggaatcaatgtaaatgcagctccattccagtccatgcaaacggtgttcaatatgaatgctccagtccctcctgctaatgaaccagaaacgttaaaacaacagagtcagtaccaggccacttataaccagagtttttccagtcagcctcaccaagtggaacaaacagagcttcaacaagaccaactgcaaacggtggttggcacttaccatggatcccaggaccagcctcatcaagtgcctggtaaccaccagcaacccccacagcagaacactggctttccacgtagcagtcagccttattacaacagtcgtggggtatctcgaggagggtctcgtggtgccagaggcttgatgaatggatacaggggccctgccaatggatttagaggaggatatgatggttaccgcccttcattctcgaacactccaaacagtggttattcacagtctcagttcactgctccccgggactactctggttaccagcgggatggatatcagcagaatttcaagcgaggctctgggcagagtggaccacggggagccccacgaggtaatatattgtggtggtgatcctagctcctatgtggagcttctgttctggccttggaagaactgttcatagtccgcatgtaggttacatgttaggaatacatttatcttttccagacttgttgctaaagattaaatgaaatgctctgtttctaaaatttcatcttgaatccaaattttaatttttgaatgactttccctgctgttgtcttcaaaatcagaacattttctctgcctcagaaaagcgtttttccaactggaaatttatttttcaggtcttaaaacctgctaaatgtttttaggaagtacctactgaaactttttgtaagacatttttggaacgagcttgaacatttatataaatttattaccctctttgatttttgaaacatgcatattatatttaggctgagaagcccttcaaatggccagataagccacagttttagctagagaaccatttagaattgacataactaatctaaacttgaacacttttaggaccaatgttagtgttctaaataccaacatatttctgatgtttaaacagatctcccaaattcttaggaccttgatgtcattaaaatttagaatgacaagcttaagaggctttagtttcatttgtttttcaagtaatgaaaaataatttcttacatgggcagatagttaatttgttgaacaattacaggtagcatttcatgtaatctgatgttctaaatggttctcttattgaaggaggttaaagaattaggtttcttacagtttttggctggccatgacatgtataaaatgtatattaaggaggaattataaagtactttaatttgaatgctagtggcaattgatcattaagaaagtactttaaagcaaaaggttaatgggtcatctgggaaaaatactgaagtatcaaaggtatttgcatgtgaatgtgggttatgttcttctatcccaccttgtagcatattctatgaaagttgagttaaatgatagctaaaatatctgtttcaacagcatgtaaaaagttattttaactgttacaagtcattatacaattttgaatgttctgtagtttctttttaacagtttaggtacaaaggtctgttttcattctggtgctttttattaattttgatagtatgatgtcacttcctattgaaatgtaagctagcgtgtaccttagaatgtgagctccatgagagcaggtaccttgtttgtcttcactgctgtatctattcccaacgcctcatgacagtgcctggcacatagtaggcactcaataaatacttgttgaatgaatgaaaaaaaaaaaaaa

SEQ ID NO: 28 - protein, 692 aa, Mus musculus; identical to SEQ ID NO: 26

SEQ ID NO: 29 - DNA, 2109 bp, Gallus gallus
  source 1..2109: mol_type = other DNA
  CDS 1..2109: protein_id = 324; translation = MPSATNGTMASSSGKAGPGGNEQAPAAAAAAPQASGGSITSVQTEAMKQILGVIDKKLRNLEKKKSKLDDYQERMNKGERLNQDQLDAVSKYQEVTNNLEFAKELQRSFMALSQDIQKTIKKTARREQLMREEAEQKRLKTVLELQFILDKLGDDEVRSDLKQGSNGVPVLTEEELTMLDEFYKLVYPERDMNMRLNEQYEQASVHLWDLLEGKEKPVCGTTYKALKEVVERILQTSYFDSTHNHQNGLCEEEEAAPTPAVEDTVAEAEPDPAEEFTEPTEVESTEYVNRQFMAETQFSSSEKEQVDEWTVETVEVVNSLQQQTQATSPPVPEPHTLTTVAQADPLVRRQRVQDLMAQMQGPYNFMQDSMLEFENQTLDPAIVSAQPMNPAQNLDMPQMVCPPVHTESRLAQPNQVPVQPEATQVPLVSSTSEGYTASQPMYQPSHTTEQRPQKESIDQIQASMSLNADQTPSSSSLPTASQPQVFQAGSSKPLHSSGINVNAAPFQSMQTVFNMNAPVPPVNEPEALKQQNQYQASYNQSFSNQPHQVEQSDLQQEQLQTVVGTYHGSPDQTHQVAGNHQQPPQQNTGFPRNSQPYYNSRGVSRGGSRGTRGLMNGYRGPANGFRGGYDGYRPSFSNTPNSGYTQPQFNAPRDYSNYQRDGYQQNFKRGSGQSGPRGAPRGRGGPPRPNRGMPQMNAQQVN
atgccctcggctaccaacggcaccatggcgagcagcagcgggaaggcgggcccgggcggcaacgagcaggccccggcggcggcagcggcggccccgcaggcgtcgggcggcagcatcacctcggttcagaccgaggccatgaagcagatcttgggagtgatcgacaaaaagctccgcaacctcgagaagaaaaagagcaaacttgacgattaccaggaacgaatgaacaagggggaacgtctaaatcaagatcaactggatgcagtgtcaaaataccaggaagtgacaaataacctggaattcgctaaagaactgcagaggagctttatggcactgagccaagatatccagaaaacaataaaaaagacggctcgcagggagcagctgatgagagaagaggctgagcagaagcgtttaaagactgtgctagagctgcagttcattttggacaagttgggtgacgatgaagtgcgcagtgacttgaaacaaggatcaaatggagtaccggtactgacagaggaggaactgacaatgctggatgaattttacaagctagtttaccctgaaagggacatgaacatgaggttgaatgagcagtatgagcaagcatctgttcacctgtgggacttactggaagggaaggaaaaacccgtttgtggaacaacctataaagccctgaaggaggttgttgaacgtattcttcaaactagttactttgatagcacccataaccatcagaacgggttatgtgaggaagaagaggcagcacccacacctgcagtagaagacactgtagcagaagctgagcctgatccagcagaagaatttactgaacctactgaagttgaatcgactgagtatgtaaacagacaattcatggcagagactcagttcagcagtagtgagaaggaacaggtagatgagtggacagttgaaacggttgaggttgtaaattcactgcagcaacaaacacaagctacatctcctccagttcctgaacctcatacactcactactgtggctcaagcagatcctcttgttagaagacagagagtacaggaccttatggcccagatgcagggtccatataacttcatgcaggactctatgctggagtttgagaaccagacacttgatcctgccattgtatctgcacagcccatgaatccagcacagaatttggacatgccgcaaatggtctgccctccagttcatactgagtcaagacttgcccagcctaatcaagttcctgtgcaaccagaagctacgcaggttcccttggtttcatctacaagtgagggatatacagcctcccagcccatgtatcagccttctcataccacagagcaacggccacagaaggaatccattgaccagattcaggcttcaatgtcactgaatgcagaccagaccccgtcatcatcatcacttcccactgcatcccagccgcaagttttccaagctggatctagcaaacctttgcatagcagcggaatcaatgttaatgcagctccattccaatccatgcaaacagtattcaacatgaatgcacctgttcctcctgttaatgagccagaagcccttaagcaacaaaatcagtaccaggccagttacaaccagagtttctccaatcagccacaccaagtagaacaatcagatcttcagcaagaacagctccagacagtggttggtacttaccatggttctccggaccagacccatcaagtggcaggaaaccaccagcaacctccccagcagaatactggatttccacgcaacagtcagccttattacaacagtcggggagtgtctcgtggtggatcacgtgggactcgtggattgatgaatggttacaggggacctgcaaatggatttagaggaggatatgatggctaccgtccttcattttccaacactccgaacagtggttacacgcagccccaatttaatgctcctcgagattattcaaactaccagcgggatggatatcagcagaacttcaaacgtggttctggacaaagtgggcctcggggagctcctcgaggtcgtggagggcccccaagaccaaacagagggatgcctcaaatgaacgctcagcaagtgaattaa

SEQ ID NO: 30 - protein, 702 aa, Gallus gallus
MPSATNGTMASSSGKAGPGGNEQAPAAAAAAPQASGGSITSVQTEAMKQILGVIDKKLRNLEKKKSKLDDYQERMNKGERLNQDQLDAVSKYQEVTNNLEFAKELQRSFMALSQDIQKTIKKTARREQLMREEAEQKRLKTVLELQFILDKLGDDEVRSDLKQGSNGVPVLTEEELTMLDEFYKLVYPERDMNMRLNEQYEQASVHLWDLLEGKEKPVCGTTYKALKEVVERILQTSYFDSTHNHQNGLCEEEEAAPTPAVEDTVAEAEPDPAEEFTEPTEVESTEYVNRQFMAETQFSSSEKEQVDEWTVETVEVVNSLQQQTQATSPPVPEPHTLTTVAQADPLVRRQRVQDLMAQMQGPYNFMQDSMLEFENQTLDPAIVSAQPMNPAQNLDMPQMVCPPVHTESRLAQPNQVPVQPEATQVPLVSSTSEGYTASQPMYQPSHTTEQRPQKESIDQIQASMSLNADQTPSSSSLPTASQPQVFQAGSSKPLHSSGINVNAAPFQSMQTVFNMNAPVPPVNEPEALKQQNQYQASYNQSFSNQPHQVEQSDLQQEQLQTVVGTYHGSPDQTHQVAGNHQQPPQQNTGFPRNSQPYYNSRGVSRGGSRGTRGLMNGYRGPANGFRGGYDGYRPSFSNTPNSGYTQPQFNAPRDYSNYQRDGYQQNFKRGSGQSGPRGAPRGRGGPPRPNRGMPQMNAQQVN

SEQ ID NO: 31 - protein, 63 aa, Homo sapiens
EEYTEQSEVESTEYVNRQFMAETQFTSGEKEQVDEWTVETVEVVNSLQQQPQAASPSVPEPHS

SEQ ID NO: 32 - protein, 18 aa, Homo sapiens
VFNMNAPVPPVNEPETLK

SEQ ID NO: 33 - protein, 16 aa, Homo sapiens
ATQVPLVSSTSEGYTA

SEQ ID NO: 34 - protein, 25 aa, Homo sapiens
QILGVIDKKLRNLEKKKGKLDDYQE

SEQ ID NO: 35 - protein, 23 aa, Homo sapiens
PRGRGGPPRPNRGMPQMNTQQVN

SEQ ID NO: 36 - protein, 5 aa, Gallus gallus
SYQMN

SEQ ID NO: 37 - protein, 17 aa, Gallus gallus
AINKFGNSTGHGAAVKG

SEQ ID NO: 38 - protein, 19 aa, Gallus gallus
HAYGYCGSGTWCAAGEIDA

SEQ ID NO: 39 - protein, 128 aa, Gallus gallus
AVTLDESGGGLQMSRGGLSLVCKASGFDFSSYQMNWIRQAPGKGLEFVAAINKFGNSTGHGAAVKGRVTISRDNGQSTVRLQLNNLRAEDTAIYFCTKHAYGYCGSGTWCAAGEIDAWGHGTEVIVSS

SEQ ID NO: 40 - protein, 9 aa, Gallus gallus
SGGGSYSYG

SEQ ID NO: 41 - protein, 7 aa, Gallus gallus
NNKRPSD

SEQ ID NO: 42 - protein, 10 aa, Gallus gallus
SGDSTDTAVF

SEQ ID NO: 43 - protein, 108 aa, Gallus gallus
QAASTQPSSVSANPGETVEITCSGGGSYSYGWFQQKSPGSAPVTVIYYNNKRPSDIPSRFSGSKSGSTGTLTITGVQADDEAVYYCGSGDSTDTAVFGAGTTLTVLGQ

SEQ ID NO: 44 - protein, 5 aa, Oryctolagus cuniculus
SHSLG

SEQ ID NO: 45 - protein, 16 aa, Oryctolagus cuniculus
DIRSGGSAYYANWAKG

SEQ ID NO: 46 - protein, 13 aa, Oryctolagus cuniculus
TNGPSDLTNRLDL

SEQ ID NO: 47 - protein, 121 aa, Homo sapiens
EQSLVESGGGLVQPGGSLRLSCAASGFSLSSHSLGWVRQAPGKGLEWIGDIRSGGSAYYANWAKGRFTISRDNSKNTLYLQMNSLRAEDTAVYYCTRTNGPSDLTNRLDLWGQGTLVTVSS

SEQ ID NO: 48 - protein, 13 aa, Oryctolagus cuniculus
QASQSLYNNENLA

SEQ ID NO: 49 - protein, 7 aa, Oryctolagus cuniculus
GASTLAS

SEQ ID NO: 50 - protein, 13 aa, Oryctolagus cuniculus
LGEFSCGSADCFA

SEQ ID NO: 51 - protein, 112 aa, Homo sapiens
QVLTQSPSSLSASVGDRVTINCQASQSLYNNENLAWFQQKPGKVPKRLIYGASTLASGVSSRFSGSGSGTEFTLTISSLQCEDFAIYYCLGEFSCGSADCFAFGGGTKVEIK

SEQ ID NO: 52 - protein, 4 aa, Gallus gallus
FDMG

SEQ ID NO: 53 - protein, 17 aa, Gallus gallus
QINDAGSRTWYATAVKG

SEQ ID NO: 54 - protein, 12 aa, Gallus gallus
GSGYVGAGAIDA

SEQ ID NO: 55 - protein, 120 aa, Gallus gallus
AVTLDESGGGLQTPGGGLSLVCKASGFTFSSFDMGWVRQAPGKGLEFVAQINDAGSRTWYATAVKGRATISRDNGQTTVRLQLNNLRAEDTGTYYCTRGSGYVGAGAIDAWGHGTEVIVS

SEQ ID NO: 56 - protein, 8 aa, Gallus gallus
SGGSGYYG

SEQ ID NO: 57 - protein, 7 aa, Gallus gallus
NDKRPSD

SEQ ID NO: 58 - protein, 10 aa, Gallus gallus
RYDSTDSGIF

SEQ ID NO: 59 - protein, 105 aa, Gallus gallus
AALTQPSSVSANPGETVKITCSGGSGYYGWYQQQKSPGSAPVTVIYQNDKRPSDIPSRFSGSGSGSTNTLTITGVQAEDEAVYFCGRYDSTDSGIFGAGTTLTVL

SEQ ID NO: 60 - protein, 6 aa, Oryctolagus cuniculus
GSYYMS

SEQ ID NO: 61 - protein, 17 aa, Oryctolagus cuniculus
YIYIGDGVTAYANWAKG

SEQ ID NO: 62 - protein, 4 aa, Oryctolagus cuniculus
GNKL

SEQ ID NO: 63 - protein, 112 aa, Oryctolagus cuniculus
QSLEESGGDLVKPGASLTLTCTASGFSFSGSYYMSWVRQAPGKGLEWIAYIYIGDGVTAYANWAKGRFTISKASSTTVTLQMTSLTAADTATYFCARGNKLWGPGTLVTVSS

SEQ ID NO: 64 - protein, 11 aa, Oryctolagus cuniculus
QASQSISSYLA

SEQ ID NO: 65 - protein, 7 aa, Oryctolagus cuniculus
DASNLDS

SEQ ID NO: 66 - protein, 14 aa, Oryctolagus cuniculus
QCTAVSSATIYGNA

SEQ ID NO: 67 - protein, 112 aa, Oryctolagus cuniculus
DVVMTQTPASVEAAVGGTVTIKCQASQSISSYLAWYQQKPGQPPKRLIYDASNLDSGVPSRFKGSGSGTDFTITISDLECADAATYYCQCTAVSSATIYGNAFGGGTEVVVK

SEQ ID NO: 68 - protein, 127 aa, Gallus gallus
AVTLDESGGGLQTPGGALSLVCKASGFTFSGYDMLWVRQAPGKGLEWVAGIGSTGGGTDYGAAVKGRATISRDNGQSTVRLQLNNLRAEDTATYYCAKVAGGCNSGYCRDSPGSIDAWGHGTEVIVS

SEQ ID NO: 69 - protein, 107 aa, Gallus gallus
AVTQQPASVSANPGETVKITCSGGGSRNYYGWYQQKSPGSVPVTVIYYDDQRPSNIPSRFSGALSGSTSTLTITGVQADDEAVYFCGSADSNTYEGSFGAGTTLTVL

SEQ ID NO: 70 - protein, 148 aa, Mus musculus
MEWSGVFIFLLSGTAGVLSEVQLHQFGAELVKPGASVKISCKASGYTFTDYNMDWVKQSHGKSLEWIGDINPNYDSTSYNQKFKGKATLTVDKSSSTAYMELRSLTSEDTAVYYCARSRSYDYEGFAYWGQGTLVTVSAAKTTPPSVY

SEQ ID NO: 71 - protein, 105 aa, Mus musculus
GLFCSVERCHYQLQSSQNLLSIVNRYHYMSGNPPKLLVYPALLIYEASITKSCVPDRFTRSGSGTNFTLTINFVHADDLIFYYCQHNRGSFLPSSSVQVPRRRSN

SEQ ID NO: 72 - protein, 109 aa, Mus musculus
PRASLGVSETLLCTSGFTFTDYYMSWVRQPPGKALEWLGFIRNKANGYTTEYSASVKGRFTISRDNSQSILYLQMNTLRAEDSATYYCARANWAFDYWGQGTTVTVSSK

SEQ ID NO: 73 - protein, 94 aa, Mus musculus
SGDRVSLSCRASQSISNYLHWYQQKSHESPRLLIKYASQSISGIPSRFSGSGSGTDFTLSINSVETEDFGMYFCQQSNSWPYTFGGGTKLEIKQ

SEQ ID NO: 74 - protein, 118 aa, Mus musculus
AAELVRPGTSVKVSCKASGYAFTNYLIVWIKQRPGQGLEWIGVISPGSGGTNYNEKFKGKAILTADKSSSTAYMQLSSLTSDEFAVYFCAREKIYDDYYEGYFDVWGAGPRHLLASLS

SEQ ID NO: 75 - protein, 107 aa, Mus musculus
GTRCDIRLTQTTSSLSASLGDRVTISCSASLGIGNYLNWYQQKPDGTVKLLIYYTSNLHSGVPSRFSGSGSGTDYSLTISNLEPEDIATYYCQHYSKLPLTFGAGPS

SEQ ID NO: 76 - protein, 113 aa, Mus musculus
GAELVRSGASVKMSCKASGYSFTDYNMYWVKQTPGQGLEWIGYIYPGNGGTNYNQKFKGKATLTADTSSSTAYMQISSLTSEDSAVYFCARDYDDGGYAMDYWGQGTTVTVSS

SEQ ID NO: 77 - protein, 117 aa, Mus musculus
LLLWLTGARCDIQMTQSPASLSASVGETVTITCRASGNIHNYLTWYQQKQGKSPQLLVYNAKTLADGVPSRFSGSGSGTQYSLKINRLQPEDFGSYYCQHFWNIPWTFGGGTKLNSR

SEQ ID NO: 78 - protein, 114 aa, Mus musculus
DAELVKPGASVKISCKASGYTFTDHSIHWVQQKPEQGLEWIGYISPGNGNIKYNEKFKGKATLTADKSSSTAYMQLNSLTSEDSAVYFCKRSLGRGGPYYFDYWGQGTTVTVSS

SEQ ID NO: 79 - protein, 108 aa, Mus musculus
DIVLTQAAPSLPVTPGESVSISCRSSKSLLHSNGNTYLYWFLQRPGQSPQLLIYRMSNLASGVPDRFSGSGSGTAFTLRISRVEAEDVGVYYCMQHREYPVTFGSGPN

SEQ ID NO: 80 - protein, 111 aa, Mus musculus
QVQLQQSGAELMKPGASVKISCKATGYTFSSYWIEWVKQRPGHGLEWIGEILPGSGSTNYNEKFKGKATFTADTSSNTAYMQLSSLTSEDSAVYYCASYYWYFDVWAQDHV

SEQ ID NO: 81 - protein, 109 aa, Mus musculus
IVMTQAAFSNPVTLGTSASISCRSSKNLLHSNGITYLYWYLQRPGQSPQLLIYRVSNLASGVPNRFSGSESGTDFTLRISRVEAEDVGVYYCAQLLELPYTSEGTKRWE

SEQ ID NO: 82 - protein, 109 aa, Mus musculus
GGGLVKPGGSLKLSCAASGFAFSSYDMSWIRQTPEKRLEWVAYISSGAGSTYYPDTVKGRFTVSRDNAKNTLYLQMSSLKSEDTAMYYCARHFYRFDYWGQGTTVTVSS

SEQ ID NO: 83 - protein, 113 aa, Mus musculus
LLLCVSGAPGSIVMTQTPKFLLVSAGDRITITCKASQSVSNDVAWYQQKPGQSPKLLIYYASNRYTGVPDRFTGSGYGTDFTFTISTVQAEDLAVYFCQQDDRFPLTFGAGPS

SEQ ID NO: 84 - protein, 112 aa, Mus musculus
QIQLVQSGPELKKPGETVKISCKASGYTFTNYGMNWVKQAPGKGLKWMGWINTYTGEPTYADDFKGRFAFSLETSASTAYLQINNLKNEDTATYFCATGAWFAYWAKDSSRH

SEQ ID NO: 85 - protein, 107 aa, Mus musculus
GVEGDIVMTQSHKFMSTSVGDRVSITCKASQDVGTAVAWYQQKPGQSPKLLIYWASTRHTGVPDRFTGSGSGTDFTLTISNVQSEDLADYFCQQYSSYPLTFGAGPS

SEQ ID NO: 86 - protein, 118 aa, Mus musculus
GGGLVQPGGSMKVSCVASGFSFIDFWMNWVRQSPEKGLEWVAEIRLKSNNYATHYAESVKGRFTISRDDSKSSVYLQMNNLRPEDTGIYYCTSLFYYYDGTSGFAYWGQGTTVTVLLK

SEQ ID NO: 87 - protein, 109 aa, Mus musculus
DIVMTQSPSSLTVTAGEKVTMHCKSSQSLLNSGDQKNYLTWYQQKPGQPPKLLIYWASTRESGVPDRFTGSGSGTDFTLTISSVQAEDLAVYYCQNDYDYPLTFGAGPS

SEQ ID NO: 88 - protein, 148 aa, Mus musculus; identical to SEQ ID NO: 70

SEQ ID NO: 89 - protein, 139 aa, Mus musculus
MSVLTQVLGLLLLWLTGARCDIQMTQSPASLSASVGETVTITCRASGNIHNYLAWYQQKQGKSPQLLVYNAKTLADGVPSRFSGSGSGTQYSLKINSLQPEDFGSYYCQHFWSTLTFGAGTKLELKRADAAPTVSNPYD

SEQ ID NO: 90 - protein, 100 aa, Mus musculus
DILQASGYSFTGYTMNWVKQSHGKNLEWIGLINPYNGGTSYNQKFKGKATLTVDKSSSTAYMELLSLTSEDSAVYYCARWGVWSAMDYWGQGTTVTVSSK

SEQ ID NO: 91 - protein, 90 aa, Mus musculus
DRVSITCKASQNVRTAVAWYQQKPRQSPKALIYLASNRDTGLPDRFPGRGSGTDFTLNITNVQSEDLEDYFCLQHCNYPNEFRGCTKVPI

SEQ ID NO: 92 - protein, 116 aa, Mus musculus
LQESGAELARPGASVKLSCKASGYTFTSYWMQWVKQRPGQGLEWIGAIYPGDGDTRYTQKFKGKATLTADKSSSTAYMQLSSLASEDSAVYYCARGEYGNYFAYWGQGTTVTVSSN

SEQ ID NO: 93 - protein, 100 aa, Mus musculus
TSDASLGERVTITCKASQDINSYLSWFQQKPGKSPKTLIYRANRLVDGVPSRFSGSGSGQDYSLTISSLEYEDMGIYYCLQYDEFPLTFGGGTKLEIKQK

SEQ ID NO: 94 - protein, 108 aa, Mus musculus
AWLSQLSCTASGFNIKDTYMHWVKQRPEQGLEWIGRIDPANGNTKYDPKFQGKATITADTSSNTAYLQLSSLTSEDTAVYYCARPIHYYYGSSLAYWGQGTTVTVSSK

SEQ ID NO: 95 - protein, 104 aa, Mus musculus
EFHAVSLGQRATISCRASESVDSYGNSFMHWYQQKPGQPPKLLIYRASNLESGIPARFSGSGSRTDFTLTINPVEADDVATYYCQQSNEDPGRSEVVPSWRSNK

SEQ ID NO: 96 - protein, 109 aa, Mus musculus; identical to SEQ ID NO: 72

SEQ ID NO: 97 - protein, 94 aa, Mus musculus; identical to SEQ ID NO: 73

SEQ ID NO: 98 - protein, 111 aa, Mus musculus
PACLPGGSLRLSCATSGFTFTDYYMSWVRQPPGKALEWLGFIRNKANGYTTEYSASVKGRFTISRDNSQSILYLQMNTLRAEDSATYYCARAPLLYYAMDYWGQGTTVTVS

SEQ ID NO: 99 - protein, 102 aa, Mus musculus
RLPFYSLEQRATISYRASKNVSTSGYSYMHWNQQKPGQPPKLLIYLVSNLESGVPARFSGSGSGTDFTLNIHPVEEEDAATYYCQHIRELTRSELVPSWKSN

SEQ ID NO: 100 - protein, 101 aa, Mus musculus
VSCKASGYTFTSYWMHWVKQRPGQGLEWIGMIDPSNSETRLNQKFKDKATLNVDKSSNTAYMQLSSLTSEDSAVYYCARGLRHYWYFDVWGQGTTVTVSSK

SEQ ID NO: 101 - protein, 99 aa, Mus musculus
TILWREGPFSYRASKSVSTSGYSYMHWNQQKPGQPPRLLIYLVSNLESGVPARFSGSGSGTDFTLNIHPVEEEDAATYYCQHIRELTRSEEVPSWRSNK

SEQ ID NO: 102 - protein, 110 aa, Mus musculus
GGGLVKPGGSLKLSCAASGFTFSSYGMSWVRQTPEKRLEWVATISSGGSYTYYPDSVKGRFTISRDNAKNTLYLQMSSLRSEDTAMYYCASLASYYFDYWGQGTTLTVSS

SEQ ID NO: 103 - protein, 113 aa, Mus musculus
GARCDVQMIQSPSSLSASLGDIVTMTCQASQGTSINLNWFQQKPGKAPKLLIYGASSLEDGVPSRFSGSCFGTDFTLTISSLEDEDMATYFCLQHSYLPPLTFGAGTKLELKR

SEQ ID NO: 104 - protein, 111 aa, Mus musculus
GPGLVQPSQSLSITCTVSGFSLTTYDLHWVRQSPGKGLEWLGVIWSGGSTDYNAAFISRLSISKDNSKSQVFFKMNSLQANDTAIYYCARNYGYSAWFAYWGQGTLVTVSA

SEQ ID NO: 105 - protein, 118 aa, Mus musculus
PASSSDVLMTQTPLSLPVSLGDQASISCRSSQSIVHSNGNTYLEWYLQKPGQSPKLLIYKVSNRFSGVPDRFSGSGSGTDFTLKISRVEAEDLGVYYCFQGSHVPLTFGAGTKLELKR

SEQ ID NO: 106 - protein, 114 aa, Mus musculus
GFELKKPGETVKISCKASGYTFTAYSMHWVKQTPGKGLKWLGWINTETGEPTYTDDFKGRFTFSLETSARIAYLQINDLKNEDTATYFCARRIYYFGRGGFDYWGQGTTVTVSS

SEQ ID NO: 107 - protein, 118 aa, Mus musculus
PASSSDVLMTQTPLSLPVRLGDQSSISCRSSQSIVHSNGNTYLEWYLQKPGQSPKLLIYKVSNRFSGVPDRFSGSGSGTDFTLKISRVEPEDLGVYYCFQGSHVPYTSEGDQAEIKLA

SEQ ID NO: 108 - protein, 114 aa, Mus musculus
GGGLVQPGGSMRLSCVASGFTFSNSWFNWVRQSPEKGLEWVAEIRLTSDNYAIYYAESVKGRFTISRDDSKSSVYLQMNNLRAEDTGIYYCTRPETARATFAYWGQGTTVTVSS

SEQ ID NO: 109 - protein, 118 aa, Mus musculus
PASTSDVLMTQTPLSLPVSLGDQASISCRSSQSIVHSNGNTYLEWYLQKPGQSPKVLIYKVFNRFSGVPDRFSGSGSGTDFTLKISRVEAEDLGVYYCFQGSHVPRTFGGGTKLNQTG

SEQ ID NO: 110 - protein, 111 aa, Mus musculus
GPDLVKPGASVKISCKASGYSFTAYYMHWVKQSHGKSLEWIGRVNPNNGGTTYNQKFKGKAILTVDKSSSTAYMELRSLTFEDSAVYYCARRIYYGYFDYWGQGTTVTVSS

SEQ ID NO: 111 - protein, 104 aa, Mus musculus
AFFAVSLGQRATISCKASQSVDYDGDSYMNWYQQKPGQPPKLLIYVASNLESGVPARFSGSGSGTDFTLNIHPVEEEDAATYYCQQSNEDPYTFGGGTKLEIKQ

SEQ ID NO: 112 - protein, 106 aa, Mus musculus
GAELVKPGASVKLSCTASGLNIRDIYMHWVKQRPEQGLEWIGKIDPANGNTKYDPKFQGKATITADTSSNTAYVQLSSLTSEDTAVYYCAGTGDYWGQGTTVTVSS

SEQ ID NO: 113 - protein, 112 aa, Mus musculus
GTCGDIVMSQSPSSLAVSAGEKVTMSCKSSQSLLNSRTRKNYLAWVQHKPGQSPRLLIYWASTRESGVPDRFTGSGSGTDFTLTISSVQAEDLAVYYCRQSYNLVTFGAGPS

SEQ ID NO: 114 - protein, 112 aa, Mus musculus
GPELVKPGASVKMSCKASGYTFTSYVMHWVKQKPGQGLEWIGYINPYNDGTKYNEKFKGKATLTSDKSSSTAYMELSSLTSEDSAVYYCARRYYYGSSGGYFDVWAQDHVRT

SEQ ID NO: 115 - protein, 108 aa, Mus musculus
DVQITQSPSYLAASPGETITINCRASKSISKYLAWYQEKPGKTNKLLIYSGSTLQSGIPSRFSGSGSGTDFTLTISSLEPEDFAMYYCQQHNEYPYTFGGGTKLEIKR

SEQ ID NO: 116 - protein, 113 aa, Mus musculus
GPELVKPGASVKISCKASGYSFTGYFMNWVMQSHGKSLEWIGRINPYNGDTFYNQKFKGKATLTVDKSSSTAHMELRSLASEDSAVYYCARRIHYYYGSSYYAMDYWGQEPHH

SEQ ID NO: 117 - protein, 108 aa, Mus musculus
DVQITQSPSYLAASPGETITINCRASKSISKYLAWYQEKPGKTNKLLIYSGSTLQSGIPSRFSGSGSGTDFTLTISSLEPEDFAMYYCQQHNEYPWTFGGGTKLEIKR

SEQ ID NO: 118 - protein, 113 aa, Mus musculus
GAGLVKPGASVKLSCKASGYTFTEYIIHWVKQRSGQGLEWIGWFYPGSGSIKYNEKFKDKATLTADKSSSTVYMELSRLTSEDSAVYFCARHEVYYDYDKSMLWTTGVKNLIR

SEQ ID NO: 119 - protein, 108 aa, Mus musculus
SPSSLAVSVGEKVTMSCKSSQSLLYSSNQKNYLAWYQQKPGQSPKLLIYWASTRESGVPDRFTGSGSGTDFTLTISSVKAEDLAVYYCQQYYSYPYTFGGGTKLEIKR

SEQ ID NO: 120 - protein, 113 aa, Mus musculus
GAELVRPGTSVKVSCKASVYAFTNYLIEWVKQRPGQGLEWIGVINPKSGGTKYNEKFRGKATLTADKSSSTAYMQLSSLTSGDSAVYFCAITGTDYWGQGTTLTVSSAKTTPP

SEQ ID NO: 121 - protein, 113 aa, Mus musculus
QGTRCDIQMTQTTSSLSASLGDRVTISCSASQGINNYLNWYQQKPDGTVKLLIYYTSSLRSGVPSRFSGSGSGTDYSLTISNLEPEDVATYYCQQYSKLPRTFGGGTKLEIKR

SEQ ID NO: 122 - protein, 121 aa, Homo sapiens
EVQLVESGGGLVQPGGSLRLSCAASGFSLSSHSLGWVRQAPGKGLEWIGDIRSGGSAYYANWAKGRFTISRDNSKNTLYLQMNSLRAEDTAVYYCTRTNGPSDLTNRLDLWGQGTLVTVSS

SEQ ID NO: 123 - protein, 112 aa, Homo sapiens; identical to SEQ ID NO: 51

SEQ ID NO: 124 - protein, 121 aa, Homo sapiens
EVQLVESGGGLVQPGGSLRLSCAASGFSLSSHSLGWVRQAPGKGLEWIGDIRSGGSAYYANWAKGRFTISRDNSKNTLYLQMNSLRAEDTAVYFCTRTNGPSDLTNRLDLWGQGTLVTVSS

SEQ ID NO: 125 - protein, 112 aa, Homo sapiens; identical to SEQ ID NO: 51

SEQ ID NO: 126 - protein, 121 aa, Homo sapiens; identical to SEQ ID NO: 122

SEQ ID NO: 127 - protein, 113 aa, Homo sapiens
EQVLTQSPSSLSASVGDRVTINCQASQSLYNNENLAWFQQKPGKVPKRLIYGASTLASGVSSRFSGSGSGTEFTLTISNLQPEDFAIYYCLGEFSCGSADCFAFGGGTKVEIK

SEQ ID NO: 128 - protein, 121 aa, Homo sapiens; identical to SEQ ID NO: 124

SEQ ID NO: 129 - protein, 113 aa, Homo sapiens
EIVLTQSPSSLSASVGDRVTINCQASQSLYNNENLAWFQQKPGKVPKRLIYGASTLASGVSSRFSGSGSGTEFTLTISNLQPEDFATYYCLGEFSCGSADCFAFGGGTKVEIK

SEQ ID NO: 130 - protein, 121 aa, Homo sapiens; identical to SEQ ID NO: 122

SEQ ID NO: 131 - protein, 113 aa, Homo sapiens; identical to SEQ ID NO: 129

SEQ ID NO: 132 - protein, 121 aa, Homo sapiens; identical to SEQ ID NO: 124

SEQ ID NO: 133 - protein, 113 aa, Homo sapiens; identical to SEQ ID NO: 127

SEQ ID NO: 134 - protein, 5 aa, Gallus gallus
GYDML

SEQ ID NO: 135 - protein, 17 aa, Gallus gallus
GIGSTGGGTDYGAAVKG

SEQ ID NO: 136 - protein, 19 aa, Gallus gallus
VAGGCNSGYCRDSPGSIDA

SEQ ID NO: 137 - protein, 10 aa, Gallus gallus
SGGGSRNYYG

SEQ ID NO: 138 - protein, 7 aa, Gallus gallus
DDQRPSN

SEQ ID NO: 139 - protein, 11 aa, Gallus gallus
SADSNTYEGSF

SEQ ID NO: 140 - protein, 5 aa, Mus musculus
DYNMD

SEQ ID NO: 141 - protein, 17 aa, Mus musculus
DINPNYDSTSYNQKFKG

SEQ ID NO: 142 - protein, 11 aa, Mus musculus
SRSYDYEGFAY

SEQ ID NO: 143 - protein, 11 aa, Mus musculus
LSIVNRYHYMS

SEQ ID NO: 144 - protein, 6 aa, Mus musculus
EASITK

SEQ ID NO: 145 - protein, 9 aa, Mus musculus
QHNRGSFLP

SEQ ID NO: 146 - protein, 5 aa, Mus musculus
DYYMS

SEQ ID NO: 147 - protein, 17 aa, Mus musculus
RNKANGYTTEYSASVKG

SEQ ID NO: 148 - protein, 9 aa, Mus musculus
ARANWAFDY

SEQ ID NO: 149 - protein, 11 aa, Mus musculus
RASQSISNYLH

SEQ ID NO: 150 - protein, 7 aa, Mus musculus
YASQSIS

SEQ ID NO: 151 - protein, 7 aa, Mus musculus
YASQSIS

SEQ ID NO: 152 - protein, 5 aa, Mus musculus
NYLIV

SEQ ID NO: 153 - protein, 17 aa, Mus musculus
VISPGSGGTNYNEKFKG

SEQ ID NO: 154 - protein, 11 aa, Mus musculus
EKIYDDYYEGY

SEQ ID NO: 155 - protein, 15 aa, Mus musculus
TISCSASLGIGNYLN

SEQ ID NO: 156 - protein, 7 aa, Mus musculus
TSNLHSG

SEQ ID NO: 157 - protein, 9 aa, Mus musculus
HYSKLPLTF

SEQ ID NO: 158 - protein, 5 aa, Mus musculus
DYNMY

SEQ ID NO: 159 - protein, 17 aa, Mus musculus
YIYPGNGGTNYNQKFKG

SEQ ID NO: 160 - protein, 11 aa, Mus musculus
DYDDGGYAMDY

SEQ ID NO: 161 - protein, 15 aa, Mus musculus
SVGETVTITCRASGN

SEQ ID NO: 162 - protein, 7 aa, Mus musculus
NAKTLAD

SEQ ID NO: 163 - protein, 9 aa, Mus musculus
QHFWNIPWT

SEQ ID NO: 164 - protein, 5 aa, Mus musculus
DHSIH

SEQ ID NO: 165 - protein, 17 aa, Mus musculus
YISPGNGNIKYNEKFKG

SEQ ID NO: 166 - protein, 12 aa, Mus musculus
SLGRGGPYYFDY

SEQ ID NO: 167 - protein, 16 aa, Mus musculus
RSSKSLLHSNGNTYLY

SEQ ID NO: 168 - protein, 7 aa, Mus musculus
RMSNLAS

SEQ ID NO: 169 - protein, 9 aa, Mus musculus
MQHREYPVT

SEQ ID NO: 170 - protein, 5 aa, Mus musculus
SYWIE

SEQ ID NO: 171 - protein, 17 aa, Mus musculus
EILPGSGSTNYNEKFKG

SEQ ID NO: 172 - protein, 11 aa, Mus musculus
YYWYFDVWAQD

SEQ ID NO: 173 - protein, 15 aa, Mus musculus
SSKNLLHSNGITYLY

SEQ ID NO: 174 - protein, 7 aa, Mus musculus
RVSNLAS

SEQ ID NO: 175 - protein, 9 aa, Mus musculus
AQLLELPYT

SEQ ID NO: 176 - protein, 5 aa, Mus musculus
SYDMS

SEQ ID NO: 177 - protein, 17 aa, Mus musculus
YISSGAGSTYYPDTVKG

SEQ ID NO: 178 - protein, 11 aa, Mus musculus
HFYRFDYWGQG

SEQ ID NO: 179 - protein, 15 aa, Mus musculus
SAGDRITITCKASQS

SEQ ID NO: 180 - protein, 7 aa, Mus musculus
YASNRYT

SEQ ID NO: 181 - protein, 9 aa, Mus musculus
QQDDRFPLT

SEQ ID NO: 182 - protein, 5 aa, Mus musculus
NYGMN

SEQ ID NO: 183 - protein, 17 aa, Mus musculus
WINTYTGEPTYADDFKG

SEQ ID NO: 184 - protein, 11 aa, Mus musculus
GAWFAYWAKDS

SEQ ID NO: 185 - protein, 15 aa, Mus musculus
SITCKASQDVGTAVA

SEQ ID NO: 186 - protein, 7 aa, Mus musculus
WASTRHT

SEQ ID NO: 187 - protein, 9 aa, Mus musculus
QQYSSYPLT

SEQ ID NO: 188 - protein, 5 aa, Mus musculus
DFWMN

SEQ ID NO: 189 - protein, 19 aa, Mus musculus
EIRLKSNNYATHYAESVKG

SEQ ID NO: 190 - protein, 13 aa, Mus musculus
LFYYYDGTSGFAY

SEQ ID NO: 191 - protein, 17 aa, Mus musculus
KSSQSLLNSGDQKNYLT

SEQ ID NO: 192 - protein, 7 aa, Mus musculus
WASTRES

SEQ ID NO: 193 - protein, 9 aa, Mus musculus
QNDYDYPLT

SEQ ID NO: 194 - protein, 5 aa, Mus musculus
DYNMD

SEQ ID NO: 195 - protein, 17 aa, Mus musculus
DINPNYDSTSYNQKFKG

SEQ ID NO: 196 - protein, 11 aa, Mus musculus
SRSYDYEGFAY

SEQ ID NO: 197 - protein, 11 aa, Mus musculus
RASGNIHNYLA

SEQ ID NO: 198 - protein, 7 aa, Mus musculus
NAKTLAD

SEQ ID NO: 199 - protein, 8 aa, Mus musculus
QHFWSTLT

SEQ ID NO: 200 - protein, 5 aa, Mus musculus
GYTMN

SEQ ID NO: 201 - protein, 16 aa, Mus musculus
NPYNGGTSYNQKFKGK

SEQ ID NO: 202 - protein, 9 aa, Mus musculus
WGVWSAMDY

SEQ ID NO: 203 - protein, 11 aa, Mus musculus
KASQNVRTAVA

SEQ ID NO: 204 - protein, 7 aa, Mus musculus
LASNRDT

SEQ ID NO: 205 - protein, 9 aa, Mus musculus
LQHCNYPNE

SEQ ID NO: 206 - protein, 5 aa, Mus musculus
SYWMQ

SEQ ID NO: 207 - protein, 17 aa, Mus musculus
AIYPGDGDTRYTQKFKG

SEQ ID NO: 208 - protein, 11 aa, Mus musculus
ARGEYGNYFAY

SEQ ID NO: 209 - protein, 11 aa, Mus musculus
KASQDINSYLS

SEQ ID NO: 210 - protein, 7 aa, Mus musculus
RANRLVD

SEQ ID NO: 211 - protein, 9 aa, Mus musculus
LQYDEFPLT

SEQ ID NO: 212 - protein, 5 aa, Mus musculus
DTYMH

SEQ ID NO: 213 - protein, 17 aa, Mus musculus
RIDPANGNTKYDPKFQG

SEQ ID NO: 214 - protein, 14 aa, Mus musculus
ARPIHYYYGSSLAY

SEQ ID NO: 215 - protein, 11 aa, Mus musculus
SVDSYGNSFMH

SEQ ID NO: 216 - protein, 7 aa, Mus musculus
RASNLES

SEQ ID NO: 217 - protein, 9 aa, Mus musculus
QQSNEDPGR

SEQ ID NO: 218 - protein, 5 aa, Mus musculus
DYYMS

SEQ ID NO: 219 - protein, 17 aa, Mus musculus
RNKANGYTTEYSASVKG

SEQ ID NO: 220 - protein, 9 aa, Mus musculus
ARANWAFDY

SEQ ID NO: 221 - protein, 11 aa, Mus musculus
RASQSISNYLH

SEQ ID NO: 222 - protein, 7 aa, Mus musculus
YASQSIS

SEQ ID NO: 223 - protein, 9 aa, Mus musculus
QQSNSWPYT

SEQ ID NO: 224 - protein, 5 aa, Mus musculus
DYYMS

SEQ ID NO: 225 - protein, 17 aa, Mus musculus
RNKANGYTTEYSASVKG

SEQ ID NO: 226 - protein, 12 aa, Mus musculus
ARAPLLYYAMDY

SEQ ID NO: 227 - protein, 11 aa, Mus musculus
NVSTSGYSYMH

SEQ ID NO: 228 - protein, 7 aa, Mus musculus
LVSNLES

SEQ ID NO: 229 - protein, 8 aa, Mus musculus
QHIRELTR

SEQ ID NO: 230 - protein, 5 aa, Mus musculus
SYWMH

SEQ ID NO: 231 - protein, 17 aa, Mus musculus
MIDPSNSETRLNQKFKD

SEQ ID NO: 232 - protein, 12 aa, Mus musculus
ARGLRHYWYFDV

SEQ ID NO: 233 - protein, 11 aa, Mus musculus
SVSTSGYSYMH

SEQ ID NO: 234 - protein, 7 aa, Mus musculus
LVSNLES

SEQ ID NO: 235 - protein, 9 aa, Mus musculus
QHIRELTRS

SEQ ID NO: 236 - protein, 5 aa, Mus musculus
SYGMS

SEQ ID NO: 237 - protein, 14 aa, Mus musculus
WVRQTPEKRLEWVA

SEQ ID NO: 238 - protein, 11 aa, Mus musculus
LASYYFDYWGQ

SEQ ID NO: 239 - protein, 15 aa, Mus musculus
TMTCQASQGTSINLN

SEQ ID NO: 240 - protein, 7 aa, Mus musculus
GASSLED

SEQ ID NO: 241 - protein, 11 aa, Mus musculus
LQHSYLPPLTF

SEQ ID NO: 242 - protein, 5 aa, Mus musculus
TYDLH

SEQ ID NO: 243 - protein, 16 aa, Mus musculus
VIWSGGSTDYNAAFIS

SEQ ID NO: 244 - protein, 11 aa, Mus musculus
NYGYSAWFAYW

SEQ ID NO: 245 - protein, 15 aa, Mus musculus
ASISCRSSQSIVHSN

SEQ ID NO: 246 - protein, 7 aa, Mus musculus
KVSNRFS

SEQ ID NO: 247 - protein, 9 aa, Mus musculus
FQGSHVPLT

SEQ ID NO: 248 - protein, 5 aa, Mus musculus
AYSMH

SEQ ID NO: 249 - protein, 17 aa, Mus musculus
WINTETGEPTYTDDFKG

SEQ ID NO: 250 - protein, 11 aa, Mus musculus
RIYYFGRGGFD

SEQ ID NO: 251 - protein, 15 aa, Mus musculus
SSISCRSSQSIVHSN

SEQ ID NO: 252 - protein, 7 aa, Mus musculus
KVSNRFS

SEQ ID NO: 253 - protein, 9 aa, Mus musculus
FQGSHVPYT

SEQ ID NO: 254 - protein, 5 aa, Mus musculus
NSWFN

SEQ ID NO: 255 - protein, 19 aa, Mus musculus
EIRLTSDNYAIYYAESVKG

SEQ ID NO: 256 - protein, 11 aa, Mus musculus
PETARATFAYW

SEQ ID NO: 257 - protein, 15 aa, Mus musculus
ASISCRSSQSIVHSN

SEQ ID NO: 258 - protein, 7 aa, Mus musculus
KVFNRFS

SEQ ID NO: 259 - protein, 9 aa, Mus musculus
FQGSHVPRT

SEQ ID NO: 260 - protein, 5 aa, Mus musculus
AYYMH

SEQ ID NO: 261 - protein, 17 aa, Mus musculus
RVNPNNGGTTYNQKFKG

SEQ ID NO: 262 - protein, 11 aa, Mus musculus
RIYYGYFDYWG

SEQ ID NO: 263 - protein, 15 aa, Mus musculus
KASQSVDYDGDSYMN

SEQ ID NO: 264 - protein, 7 aa, Mus musculus
VASNLES

SEQ ID NO: 265 - protein, 9 aa, Mus musculus
QQSNEDPYT

SEQ ID NO: 266 - protein, 4 aa, Mus musculus
DIYM

SEQ ID NO: 267 - protein, 17 aa, Mus musculus
KIDPANGNTKYDPKFQG

SEQ ID NO: 268 - protein, 11 aa, Mus musculus
TGDYWGQGTTV

SEQ ID NO: 269 - protein, 15 aa, Mus musculus
TMSCKSSQSLLNSRT

SEQ ID NO: 270 - protein, 7 aa, Mus musculus
WASTRES

SEQ ID NO: 271 - protein, 9 aa, Mus musculus
RQSYNLVTF

SEQ ID NO: 272 - protein, 5 aa, Mus musculus
SYVMH

SEQ ID NO: 273 - protein, 17 aa, Mus musculus
YINPYNDGTKYNEKFKG

SEQ ID NO: 274 - protein, 11 aa, Mus musculus
RYYYGSSGGYF

SEQ ID NO: 275 - protein, 15 aa, Mus musculus
RASKSISKYLAWYQE

SEQ ID NO: 276 - protein, 7 aa, Mus musculus
SGSTLQS

SEQ ID NO: 277 - protein, 9 aa, Mus musculus
QQHNEYPYT

SEQ ID NO: 278 - protein, 5 aa, Mus musculus
GYFMN

SEQ ID NO: 279 - protein, 17 aa, Mus musculus
RINPYNGDTFYNQKFKG

SEQ ID NO: 280 - protein, 11 aa, Mus musculus
RIHYYYGSSYY

SEQ ID NO: 281 - protein, 15 aa, Mus musculus
RASKSISKYLAWYQE

SEQ ID NO: 282 - protein, 7 aa, Mus musculus
SGSTLQS

SEQ ID NO: 283 - protein, 9 aa, Mus musculus
QQHNEYPWT

SEQ ID NO: 284 - protein, 5 aa, Mus musculus
EYIIH

SEQ ID NO: 285 - protein, 17 aa, Mus musculus
WFYPGSGSIKYNEKFKD

SEQ ID NO: 286 - protein, 11 aa, Mus musculus
HEVYYDYDKSM

SEQ ID NO: 287 - protein, 15 aa, Mus musculus
LYSSNQKNYLAWYQQ

SEQ ID NO: 288 - protein, 7 aa, Mus musculus
WASTRES

SEQ ID NO: 289 - protein, 9 aa, Mus musculus
QQYYSYPYT

SEQ ID NO: 290 - protein, 5 aa, Mus musculus
NYLIE

SEQ ID NO: 291 - protein, 19 aa, Mus musculus
VINPKSGGTKYNEKFRGKA

SEQ ID NO: 292 - protein, 11 aa, Mus musculus
TGTDYWGQGTT

SEQ ID NO: 293 - protein, 10 aa, Mus musculus
VTISCSASQG

SEQ ID NO: 294 - protein, 7 aa, Mus musculus
YTSSLRS

SEQ ID NO: 295 - protein, 9 aa, Mus musculus
QQYSKLPRT

SEQ ID NO: 296 - protein, 12 aa, Homo sapiens
FTSGEKEQVDEW

SEQ ID NO: 297 - protein, 16 aa, Homo sapiens
AEQKRLKTVLELQYVL

SEQ ID NO: 298 - protein, 16 aa, Homo sapiens
VERVFQSNYFDSTHNH

SEQ ID NO: 299 - protein, 16 aa, Homo sapiens
FQSMQTVFNMNAPVPP

SEQ ID NO: 300 - protein, 5 aa, Mus musculus
TNAMN

SEQ ID NO: 301 - protein, 17 aa, Mus musculus
RIRSKSNNYATYYADSV

SEQ ID NO: 302 - protein, 11 aa, Mus musculus
DWDGFLYFDYW

SEQ ID NO: 303 - protein, 112 aa, Mus musculus
GGGLVQPKGSLKLSCAASGFTFNTNAMNWVRQAPGKGLEWVARIRSKSNNYATYYADSVKDRFTISRDDSQSMLYLQMNNLKTEDTAMYYCVRDWDGFLYFDYWAKHHLTLF

SEQ ID NO: 304 - protein, 15 aa, Mus musculus
SVSTSGYSYMHWNQQ

SEQ ID NO: 305 - protein, 7 aa, Mus musculus
LVSNLES

SEQ ID NO: 306 - protein, 9 aa, Mus musculus
QHIRELTRS

SEQ ID NO: 307 - protein, 104 aa, Mus musculus
TQSPASLAVSLGQRATISYRASKSVSTSGYSYMHWNQQKPGQPPRLLIYLVSNLESGVPARFSGSGSGTDFTLNIHPVEEEDAATYYCQHIRELTRSEGGPSWK

SEQ ID NO: 308 - protein, 14 aa, Homo sapiens
PPVNEPETLKQQNQ

SEQ ID NO: 309 - protein, 12 aa, Homo sapiens
ETLKQQNQYQAS

SEQ ID NO: 310 - protein, 709 aa, Homo sapiens; identical to SEQ ID NO: 2

SEQ ID NO: 311 - protein, 694 aa, Homo sapiens; identical to SEQ ID NO: 4

SEQ ID NO: 312 - protein, 448 aa, Canis familiaris; identical to SEQ ID NO: 6

SEQ ID NO: 313 - protein, 717 aa, Canis familiaris; identical to SEQ ID NO: 8

SEQ ID NO: 314 - protein, 702 aa, Canis familiaris; identical to SEQ ID NO: 10

SEQ ID NO: 315 - protein, 679 aa, Canis familiaris; identical to SEQ ID NO: 12

SEQ ID NO: 316 - protein, 717 aa, Canis familiaris; identical to SEQ ID NO: 8

SEQ ID NO: 317 - protein, 708 aa, Bos taurus; identical to SEQ ID NO: 16

SEQ ID NO: 318 - protein, 638 aa, Equus caballus; identical to SEQ ID NO: 18

SEQ ID NO: 319 - protein, 707 aa, Mus musculus; identical to SEQ ID NO: 20

SEQ ID NO: 320 - protein, 707 aa, Mus musculus; identical to SEQ ID NO: 20

SEQ ID NO: 321 - protein, 698 aa, Mus musculus; identical to SEQ ID NO: 24

SEQ ID NO: 322 - protein, 692 aa, Mus musculus; identical to SEQ ID NO: 26

SEQ ID NO: 323 - protein, 692 aa, Mus musculus; identical to SEQ ID NO: 26

SEQ ID NO: 324 - protein, 702 aa, Gallus gallus; identical to SEQ ID NO: 30